European Patent Application EP 4 151 659 A1, published March 22, 2023. Title: 生物大分子靶向特异性补体抑制剂及其制备方法与应用. Applicant: 上海康景生物医药科技有限公司. The sequence listing filed with the application follows.

SEQUENCE LISTING (68 sequences)

SEQ ID NO: 1 - DNA, 1200 bp, 人类（Homo sapiens）
atggggatcttactgggcctgctactcctggggcacctaacagtggacacttatggccgtcccatcctggaagtgccagagagtgtaacaggaccttggaaaggggatgtgaatcttccctgcacctatgaccccctgcaaggctacacccaagtcttggtgaagtggctggtacaacgtggctcagaccctgtcaccatctttctacgtgactcttctggagaccatatccagcaggcaaagtaccagggccgcctgcatgtgagccacaaggttccaggagatgtatccctccaattgagcaccctggagatggatgaccggagccactacacgtgtgaagtcacctggcagactcctgatggcaaccaagtcgtgagagataagattactgagctccgtgtccagaaactctctgtctccaagcccacagtgacaactggcagcggttatggcttcacggtgccccagggaatgaggattagccttcaatgccaggctcggggttctcctcccatcagttatatttggtataagcaacagactaataaccaggaacccatcaaagtagcaaccctaagtaccttactcttcaagcctgcggtgatagccgactcaggctcctatttctgcactgccaagggccaggttggctctgagcagcacagcgacattgtgaagtttgtggtcaaagactcctcaaagctactcaagaccaagactgaggcacctacaaccatgacataccccttgaaagcaacatctacagtgaagcagtcctgggactggaccactgacatggatggctaccttggagagaccagtgctgggccaggaaagagcctgcctgtctttgccatcatcctcatcatctccttgtgctgtatggtggtttttaccatggcctatatcatgctctgtcggaagacatcccaacaagagcatgtctacgaagcagccagggcacatgccagagaggccaacgactctggagaaaccatgagggtggccatcttcgcaagtggctgctccagtgatgagccaacttcccagaatctgggcaacaactactctgatgagccctgcataggacaggagtaccagatcatcgcccagatcaatggcaactacgcccgcctgctggacacagttcctctggattatgagtttctggccactgagggcaaaagtgtctgttaa

SEQ ID NO: 2 - protein, 399 aa, 人类（Homo sapiens）
MGILLGLLLLGHLTVDTYGRPILEVPESVTGPWKGDVNLPCTYDPLQGYTQVLVKWLVQRGSDPVTIFLRDSSGDHIQQAKYQGRLHVSHKVPGDVSLQLSTLEMDDRSHYTCEVTWQTPDGNQVVRDKITELRVQKLSVSKPTVTTGSGYGFTVPQGMRISLQCQARGSPPISYIWYKQQTNNQEPIKVATLSTLLFKPAVIADSGSYFCTAKGQVGSEQHSDIVKFVVKDSSKLLKTKTEAPTTMTYPLKATSTVKQSWDWTTDMDGYLGETSAGPGKSLPVFAIILIISLCCMVVFTMAYIMLCRKTSQQEHVYEAARAHAREANDSGETMRVAIFASGCSSDEPTSQNLGNNYSDEPCIGQEYQIIAQINGNYARLLDTVPLDYEFLATEGKSVC

SEQ ID NO: 3 - DNA, 3696 bp, 人类（Homo sapiens）
atgagacttctagcaaagattatttgccttatgttatgggctatttgtgtagcagaagattgcaatgaacttcctccaagaagaaatacagaaattctgacaggttcctggtctgaccaaacatatccagaaggcacccaggctatctataaatgccgccctggatatagatctcttggaaatgtaataatggtatgcaggaagggagaatgggttgctcttaatccattaaggaaatgtcagaaaaggccctgtggacatcctggagatactccttttggtacttttacccttacaggaggaaatgtgtttgaatatggtgtaaaagctgtgtatacatgtaatgaggggtatcaattgctaggtgagattaattaccgtgaatgtgacacagatggatggaccaatgatattcctatatgtgaagttgtgaagtgtttaccagtgacagcaccagagaatggaaaaattgtcagtagtgcaatggaaccagatcgggaataccattttggacaagcagtacggtttgtatgtaactcaggctacaagattgaaggagatgaagaaatgcattgttcagacgatggtttttggagtaaagagaaaccaaagtgtgtggaaatttcatgcaaatccccagatgttataaatggatctcctatatctcagaagattatttataaggagaatgaacgatttcaatataaatgtaacatgggttatgaatacagtgaaagaggagatgctgtatgcactgaatctggatggcgtccgttgccttcatgtgaagaaaaatcatgtgataatccttatattccaaatggtgactactcacctttaaggattaaacacagaactggagatgaaatcacgtaccagtgtagaaatggtttttatcctgcaacccggggaaatacagcaaaatgcacaagtactggctggatacctgctccgagatgtaccttgaaaccttgtgattatccagacattaaacatggaggtctatatcatgagaatatgcgtagaccatactttccagtagctgtaggaaaatattactcctattactgtgatgaacattttgagactccgtcaggaagttactgggatcacattcattgcacacaagatggatggtcgccagcagtaccatgcctcagaaaatgttattttccttatttggaaaatggatataatcaaaatcatggaagaaagtttgtacagggtaaatctatagacgttgcctgccatcctggctacgctcttccaaaagcgcagaccacagttacatgtatggagaatggctggtctcctactcccagatgcatccgtgtcaaaacatgttccaaatcaagtatagatattgagaatgggtttatttctgaatctcagtatacatatgccttaaaagaaaaagcgaaatatcaatgcaaactaggatatgtaacagcagatggtgaaacatcaggatcaattacatgtgggaaagatggatggtcagctcaacccacgtgcattaaatcttgtgatatcccagtatttatgaatgccagaactaaaaatgacttcacatggtttaagctgaatgacacattggactatgaatgccatgatggttatgaaagcaatactggaagcaccactggttccatagtgtgtggttacaatggttggtctgatttacccatatgttatgaaagagaatgcgaacttcctaaaatagatgtacacttagttcctgatcgcaagaaagaccagtataaagttggagaggtgttgaaattctcctgcaaaccaggatttacaatagttggacctaattccgttcagtgctaccactttggattgtctcctgacctcccaatatgtaaagagcaagtacaatcatgtggtccacctcctgaactcctcaatgggaatgttaaggaaaaaacgaaagaagaatatggacacagtgaagtggtggaatattattgcaatcctagatttctaatgaagggacctaataaaattcaatgtgttgatggagagtggacaactttaccagtgtgtattgtggaggagagtacctgtggagatatacctgaacttgaacatggctgggcccagctttcttcccctccttattactatggagattcagtggaattcaattgctcagaatcatttacaatgattggacacagatcaattacgtgtattcatggagtatggacccaacttccccagtgtgtggcaatagataaacttaagaagtgcaaatcatcaaatttaattatacttgaggaacatttaaaaaacaagaaggaattcgatcataattctaacataaggtacagatgtagaggaaaagaaggatggatacacacagtctgcataaatggaagatgggatccagaagtgaactgctcaatggcacaaatacaattatgcccacctccacctcagattcccaattctcacaatatgacaaccacactgaattatcgggatggagaaaaagtatctgttctttgccaagaaaattatctaattcaggaaggagaagaaattacatgcaaagatggaagatggcagtcaataccactctgtgttgaaaaaattccatgttcacaaccacctcagatagaacacggaaccattaattcatccaggtcttcacaagaaagttatgcacatgggactaaattgagttatacttgtgagggtggtttcaggatatctgaagaaaatgaaacaacatgctacatgggaaaatggagttctccacctcagtgtgaaggccttccttgtaaatctccacctgagatttctcatggtgttgtagctcacatgtcagacagttatcagtatggagaagaagttacgtacaaatgttttgaaggttttggaattgatgggcctgcaattgcaaaatgcttaggagaaaaatggtctcaccctccatcatgcataaaaacagattgtctcagtttacctagctttgaaaatgccatacccatgggagagaagaaggatgtgtataaggcgggtgagcaagtgacttacacttgtgcaacatattacaaaatggatggagccagtaatgtaacatgcattaatagcagatggacaggaaggccaacatgcagagacacctcctgtgtgaatccgcccacagtacaaaatgcttatatagtgtcgagacagatgagtaaatatccatctggtgagagagtacgttatcaatgtaggagcccttatgaaatgtttggggatgaagaagtgatgtgtttaaatggaaactggacggaaccacctcaatgcaaagattctacaggaaaatgtgggccccctccacctattgacaatggggacattacttcattcccgttgtcagtatatgctccagcttcatcagttgagtaccaatgccagaacttgtatcaacttgagggtaacaagcgaataacatgtagaaatggacaatggtcagaaccaccaaaatgcttacatccgtgtgtaatatcccgagaaattatggaaaattataacatagcattaaggtggacagccaaacagaagctttattcgagaacaggtgaatcagttgaatttgtgtgtaaacggggatatcgtctttcatcacgttctcacacattgcgaacaacatgttgggatgggaaactggagtatccaacttgtgcaaaaagatag

SEQ ID NO: 4 - protein, 1231 aa, 人类（Homo sapiens）
MRLLAKIICLMLWAICVAEDCNELPPRRNTEILTGSWSDQTYPEGTQAIYKCRPGYRSLGNVIMVCRKGEWVALNPLRKCQKRPCGHPGDTPFGTFTLTGGNVFEYGVKAVYTCNEGYQLLGEINYRECDTDGWTNDIPICEVVKCLPVTAPENGKIVSSAMEPDREYHFGQAVRFVCNSGYKIEGDEEMHCSDDGFWSKEKPKCVEISCKSPDVINGSPISQKIIYKENERFQYKCNMGYEYSERGDAVCTESGWRPLPSCEEKSCDNPYIPNGDYSPLRIKHRTGDEITYQCRNGFYPATRGNTAKCTSTGWIPAPRCTLKPCDYPDIKHGGLYHENMRRPYFPVAVGKYYSYYCDEHFETPSGSYWDHIHCTQDGWSPAVPCLRKCYFPYLENGYNQNHGRKFVQGKSIDVACHPGYALPKAQTTVTCMENGWSPTPRCIRVKTCSKSSIDIENGFISESQYTYALKEKAKYQCKLGYVTADGETSGSITCGKDGWSAQPTCIKSCDIPVFMNARTKNDFTWFKLNDTLDYECHDGYESNTGSTTGSIVCGYNGWSDLPICYERECELPKIDVHLVPDRKKDQYKVGEVLKFSCKPGFTIVGPNSVQCYHFGLSPDLPICKEQVQSCGPPPELLNGNVKEKTKEEYGHSEVVEYYCNPRFLMKGPNKIQCVDGEWTTLPVCIVEESTCGDIPELEHGWAQLSSPPYYYGDSVEFNCSESFTMIGHRSITCIHGVWTQLPQCVAIDKLKKCKSSNLIILEEHLKNKKEFDHNSNIRYRCRGKEGWIHTVCINGRWDPEVNCSMAQIQLCPPPPQIPNSHNMTTTLNYRDGEKVSVLCQENYLIQEGEEITCKDGRWQSIPLCVEKIPCSQPPQIEHGTINSSRSSQESYAHGTKLSYTCEGGFRISEENETTCYMGKWSSPPQCEGLPCKSPPEISHGVVAHMSDSYQYGEEVTYKCFEGFGIDGPAIAKCLGEKWSHPPSCIKTDCLSLPSFENAIPMGEKKDVYKAGEQVTYTCATYYKMDGASNVTCINSRWTGRPTCRDTSCVNPPTVQNAYIVSRQMSKYPSGERVRYQCRSPYEMFGDEEVMCLNGNWTEPPQCKDSTGKCGPPPPIDNGDITSFPLSVYAPASSVEYQCQNLYQLEGNKRITCRNGQWSEPPKCLHPCVISREIMENYNIALRWTAKQKLYSRTGESVEFVCKRGYRLSSRSHTLRTTCWDGKLEYPTCAKR

SEQ ID NO: 5 - DNA, 357 bp, 人类（Homo sapiens）
ggccgtcccatcctggaagtgccagagagtgtaacaggaccttggaaaggggatgtgaatcttccctgcacctatgaccccctgcaaggctacacccaagtcttggtgaagtggctggtacaacgtggctcagaccctgtcaccatctttctacgtgactcttctggagaccatatccagcaggcaaagtaccagggccgcctgcatgtgagccacaaggttccaggagatgtatccctccaattgagcaccctggagatggatgaccggagccactacacgtgtgaagtcacctggcagactcctgatggcaaccaagtcgtgagagataagattactgagctccgtgtccagaaa

SEQ ID NO: 6 - protein, 119 aa, 人类（Homo sapiens）
GRPILEVPESVTGPWKGDVNLPCTYDPLQGYTQVLVKWLVQRGSDPVTIFLRDSSGDHIQQAKYQGRLHVSHKVPGDVSLQLSTLEMDDRSHYTCEVTWQTPDGNQVVRDKITELRVQK

SEQ ID NO: 7 - DNA, 915 bp, 人类（Homo sapiens）
gaagattgcaatgaacttcctccaagaagaaatacagaaattctgacaggttcctggtctgaccaaacatatccagaaggcacccaggctatctataaatgccgccctggatatagatctcttggaaatgtaataatggtatgcaggaagggagaatgggttgctcttaatccattaaggaaatgtcagaaaaggccctgtggacatcctggagatactccttttggtacttttacccttacaggaggaaatgtgtttgaatatggtgtaaaagctgtgtatacatgtaatgaggggtatcaattgctaggtgagattaattaccgtgaatgtgacacagatggatggaccaatgatattcctatatgtgaagttgtgaagtgtttaccagtgacagcaccagagaatggaaaaattgtcagtagtgcaatggaaccagatcgggaataccattttggacaagcagtacggtttgtatgtaactcaggctacaagattgaaggagatgaagaaatgcattgttcagacgatggtttttggagtaaagagaaaccaaagtgtgtggaaatttcatgcaaatccccagatgttataaatggatctcctatatctcagaagattatttataaggagaatgaacgatttcaatataaatgtaacatgggttatgaatacagtgaaagaggagatgctgtatgcactgaatctggatggcgtccgttgccttcatgtgaagaaaaatcatgtgataatccttatattccaaatggtgactactcacctttaaggattaaacacagaactggagatgaaatcacgtaccagtgtagaaatggtttttatcctgcaacccggggaaatacagcaaaatgcacaagtactggctggatacctgctccgagatgtaccttgaaa

SEQ ID NO: 8 - protein, 305 aa, 人类（Homo sapiens）
EDCNELPPRRNTEILTGSWSDQTYPEGTQAIYKCRPGYRSLGNVIMVCRKGEWVALNPLRKCQKRPCGHPGDTPFGTFTLTGGNVFEYGVKAVYTCNEGYQLLGEINYRECDTDGWTNDIPICEVVKCLPVTAPENGKIVSSAMEPDREYHFGQAVRFVCNSGYKIEGDEEMHCSDDGFWSKEKPKCVEISCKSPDVINGSPISQKIIYKENERFQYKCNMGYEYSERGDAVCTESGWRPLPSCEEKSCDNPYIPNGDYSPLRIKHRTGDEITYQCRNGFYPATRGNTAKCTSTGWIPAPRCTLK

SEQ ID NO: 9 - DNA, 675 bp, 人类（Homo sapiens）
cccccatgcccatcatgcccagcacctgagttcctggggggaccatcagtcttcctgttccccccaaaacccaaggacactctcatgatctcccggacccctgaggtcacgtgcgtggtggtggacgtgagccaggaagaccccgaggtccagttcaactggtacgtggatggcgtggaggtgcataatgccaagacaaagccgcgggaggagcagttcaacagcacgtaccgtgtggtcagcgtcctcaccgtcctgcaccaggactggctgaacggcaaggagtacaagtgcaaggtctccaacaaaggcctcccgtcctccatcgagaaaaccatctccaaagccaaagggcagccccgagagccacaggtgtacaccctgcccccatcccaggaggagatgaccaagaaccaggtcagcctgacctgcctggtcaaaggcttctaccccagcgacatcgccgtggagtgggagagcaatgggcagccggagaacaactacaagaccacgcctcccgtgctggactccgacggctccttcttcctctacagcaggctaaccgtggacaagagcaggtggcaggaggggaatgtcttctcatgctccgtgatgcatgaggctctgcacaaccactacacacagaagagcctctccctgtctctgggtaaataa

SEQ ID NO: 10 - protein, 224 aa, 人类（Homo sapiens）
PPCPSCPAPEFLGGPSVFLFPPKPKDTLMISRTPEVTCVVVDVSQEDPEVQFNWYVDGVEVHNAKTKPREEQFNSTYRVVSVLTVLHQDWLNGKEYKCKVSNKGLPSSIEKTISKAKGQPREPQVYTLPPSQEEMTKNQVSLTCLVKGFYPSDIAVEWESNGQPENNYKTTPPVLDSDGSFFLYSRLTVDKSRWQEGNVFSCSVMHEALHNHYTQKSLSLSLGK

SEQ ID NO: 11 - DNA, 1758 bp, 人类（Homo sapiens）
gatgcacacaagagtgaggttgctcatcggtttaaagatttgggagaagaaaatttcaaagccttggtgttgattgcctttgctcagtatcttcagcagtgtccatttgaagatcatgtaaaattagtgaatgaagtaactgaatttgcaaaaacatgtgttgctgatgagtcagctgaaaattgtgacaaatcacttcataccctttttggagacaaattatgcacagttgcaactcttcgtgaaacctatggtgaaatggctgactgctgtgcaaaacaagaacctgagagaaatgaatgcttcttgcaacacaaagatgacaacccaaacctcccccgattggtgagaccagaggttgatgtgatgtgcactgcttttcatgacaatgaagagacatttttgaaaaaatacttatatgaaattgccagaagacatccttacttttatgccccggaactccttttctttgctaaaaggtataaagctgcttttacagaatgttgccaagctgctgataaagctgcctgcctgttgccaaagctcgatgaacttcgggatgaagggaaggcttcgtctgccaaacagagactcaagtgtgccagtctccaaaaatttggagaaagagctttcaaagcatgggcagtagctcgcctgagccagagatttcccaaagctgagtttgcagaagtttccaagttagtgacagatcttaccaaagtccacacggaatgctgccatggagatctgcttgaatgtgctgatgacagggcggaccttgccaagtatatctgtgaaaatcaagattcgatctccagtaaactgaaggaatgctgtgaaaaacctctgttggaaaaatcccactgcattgccgaagtggaaaatgatgagatgcctgctgacttgccttcattagctgctgattttgttgaaagtaaggatgtttgcaaaaactatgctgaggcaaaggatgtcttcctgggcatgtttttgtatgaatatgcaagaaggcatcctgattactctgtcgtgctgctgctgagacttgccaagacatatgaaaccactctagagaagtgctgtgccgctgcagatcctcatgaatgctatgccaaagtgttcgatgaatttaaacctcttgtggaagagcctcagaatttaatcaaacaaaattgtgagctttttgagcagcttggagagtacaaattccagaatgcgctattagttcgttacaccaagaaagtaccccaagtgtcaactccaactcttgtagaggtctcaagaaacctaggaaaagtgggcagcaaatgttgtaaacatcctgaagcaaaaagaatgccctgtgcagaagactatctatccgtggtcctgaaccagttatgtgtgttgcatgagaaaacgccagtaagtgacagagtcaccaaatgctgcacagaatccttggtgaacaggcgaccatgcttttcagctctggaagtcgatgaaacatacgttcccaaagagtttaatgctgaaacattcaccttccatgcagatatatgcacactttctgagaaggagagacaaatcaagaaacaaactgcacttgttgagctcgtgaaacacaagcccaaggcaacaaaagagcaactgaaagctgttatggatgatttcgcagcttttgtagagaagtgctgcaaggctgacgataaggagacctgctttgccgaggagggtaaaaaacttgttgctgcaagtcaagctgccttaggcttataa

SEQ ID NO: 12 - protein, 585 aa, 人类（Homo sapiens） [sequence omitted]

SEQ ID NO: 13 - DNA, 1950 bp, 人工序列（Artificial Sequence）
  CRIg-FH-IgG4 Fc核酸序列
atgggccgtcccatcctggaagtgccagagagtgtaacaggaccttggaaaggggatgtgaatcttccctgcacctatgaccccctgcaaggctacacccaagtcttggtgaagtggctggtacaacgtggctcagaccctgtcaccatctttctacgtgactcttctggagaccatatccagcaggcaaagtaccagggccgcctgcatgtgagccacaaggttccaggagatgtatccctccaattgagcaccctggagatggatgaccggagccactacacgtgtgaagtcacctggcagactcctgatggcaaccaagtcgtgagagataagattactgagctccgtgtccagaaagaagattgcaatgaacttcctccaagaagaaatacagaaattctgacaggttcctggtctgaccaaacatatccagaaggcacccaggctatctataaatgccgccctggatatagatctcttggaaatgtaataatggtatgcaggaagggagaatgggttgctcttaatccattaaggaaatgtcagaaaaggccctgtggacatcctggagatactccttttggtacttttacccttacaggaggaaatgtgtttgaatatggtgtaaaagctgtgtatacatgtaatgaggggtatcaattgctaggtgagattaattaccgtgaatgtgacacagatggatggaccaatgatattcctatatgtgaagttgtgaagtgtttaccagtgacagcaccagagaatggaaaaattgtcagtagtgcaatggaaccagatcgggaataccattttggacaagcagtacggtttgtatgtaactcaggctacaagattgaaggagatgaagaaatgcattgttcagacgatggtttttggagtaaagagaaaccaaagtgtgtggaaatttcatgcaaatccccagatgttataaatggatctcctatatctcagaagattatttataaggagaatgaacgatttcaatataaatgtaacatgggttatgaatacagtgaaagaggagatgctgtatgcactgaatctggatggcgtccgttgccttcatgtgaagaaaaatcatgtgataatccttatattccaaatggtgactactcacctttaaggattaaacacagaactggagatgaaatcacgtaccagtgtagaaatggtttttatcctgcaacccggggaaatacagcaaaatgcacaagtactggctggatacctgctccgagatgtaccttgaaacccccatgcccatcatgcccagcacctgagttcctggggggaccatcagtcttcctgttccccccaaaacccaaggacactctcatgatctcccggacccctgaggtcacgtgcgtggtggtggacgtgagccaggaagaccccgaggtccagttcaactggtacgtggatggcgtggaggtgcataatgccaagacaaagccgcgggaggagcagttcaacagcacgtaccgtgtggtcagcgtcctcaccgtcctgcaccaggactggctgaacggcaaggagtacaagtgcaaggtctccaacaaaggcctcccgtcctccatcgagaaaaccatctccaaagccaaagggcagccccgagagccacaggtgtacaccctgcccccatcccaggaggagatgaccaagaaccaggtcagcctgacctgcctggtcaaaggcttctaccccagcgacatcgccgtggagtgggagagcaatgggcagccggagaacaactacaagaccacgcctcccgtgctggactccgacggctccttcttcctctacagcaggctaaccgtggacaagagcaggtggcaggaggggaatgtcttctcatgctccgtgatgcatgaggctctgcacaaccactacacacagaagagcctctccctgtctctgggtaaataa

SEQ ID NO: 14 - protein, 649 aa, 人工序列（Artificial Sequence）
  CRIg-FH-IgG4 Fc蛋白序列
MGRPILEVPESVTGPWKGDVNLPCTYDPLQGYTQVLVKWLVQRGSDPVTIFLRDSSGDHIQQAKYQGRLHVSHKVPGDVSLQLSTLEMDDRSHYTCEVTWQTPDGNQVVRDKITELRVQKEDCNELPPRRNTEILTGSWSDQTYPEGTQAIYKCRPGYRSLGNVIMVCRKGEWVALNPLRKCQKRPCGHPGDTPFGTFTLTGGNVFEYGVKAVYTCNEGYQLLGEINYRECDTDGWTNDIPICEVVKCLPVTAPENGKIVSSAMEPDREYHFGQAVRFVCNSGYKIEGDEEMHCSDDGFWSKEKPKCVEISCKSPDVINGSPISQKIIYKENERFQYKCNMGYEYSERGDAVCTESGWRPLPSCEEKSCDNPYIPNGDYSPLRIKHRTGDEITYQCRNGFYPATRGNTAKCTSTGWIPAPRCTLKPPCPSCPAPEFLGGPSVFLFPPKPKDTLMISRTPEVTCVVVDVSQEDPEVQFNWYVDGVEVHNAKTKPREEQFNSTYRVVSVLTVLHQDWLNGKEYKCKVSNKGLPSSIEKTISKAKGQPREPQVYTLPPSQEEMTKNQVSLTCLVKGFYPSDIAVEWESNGQPENNYKTTPPVLDSDGSFFLYSRLTVDKSRWQEGNVFSCSVMHEALHNHYTQKSLSLSLGK

SEQ ID NO: 15 - DNA, 3030 bp, 人工序列（Artificial Sequence）
  CRIg-FH-HSA核酸序列
ggccgtcccatcctggaagtgccagagagtgtaacaggaccttggaaaggggatgtgaatcttccctgcacctatgaccccctgcaaggctacacccaagtcttggtgaagtggctggtacaacgtggctcagaccctgtcaccatctttctacgtgactcttctggagaccatatccagcaggcaaagtaccagggccgcctgcatgtgagccacaaggttccaggagatgtatccctccaattgagcaccctggagatggatgaccggagccactacacgtgtgaagtcacctggcagactcctgatggcaaccaagtcgtgagagataagattactgagctccgtgtccagaaagaagattgcaatgaacttcctccaagaagaaatacagaaattctgacaggttcctggtctgaccaaacatatccagaaggcacccaggctatctataaatgccgccctggatatagatctcttggaaatgtaataatggtatgcaggaagggagaatgggttgctcttaatccattaaggaaatgtcagaaaaggccctgtggacatcctggagatactccttttggtacttttacccttacaggaggaaatgtgtttgaatatggtgtaaaagctgtgtatacatgtaatgaggggtatcaattgctaggtgagattaattaccgtgaatgtgacacagatggatggaccaatgatattcctatatgtgaagttgtgaagtgtttaccagtgacagcaccagagaatggaaaaattgtcagtagtgcaatggaaccagatcgggaataccattttggacaagcagtacggtttgtatgtaactcaggctacaagattgaaggagatgaagaaatgcattgttcagacgatggtttttggagtaaagagaaaccaaagtgtgtggaaatttcatgcaaatccccagatgttataaatggatctcctatatctcagaagattatttataaggagaatgaacgatttcaatataaatgtaacatgggttatgaatacagtgaaagaggagatgctgtatgcactgaatctggatggcgtccgttgccttcatgtgaagaaaaatcatgtgataatccttatattccaaatggtgactactcacctttaaggattaaacacagaactggagatgaaatcacgtaccagtgtagaaatggtttttatcctgcaacccggggaaatacagcaaaatgcacaagtactggctggatacctgctccgagatgtaccttgaaagatgcacacaagagtgaggttgctcatcggtttaaagatttgggagaagaaaatttcaaagccttggtgttgattgcctttgctcagtatcttcagcagtgtccatttgaagatcatgtaaaattagtgaatgaagtaactgaatttgcaaaaacatgtgttgctgatgagtcagctgaaaattgtgacaaatcacttcataccctttttggagacaaattatgcacagttgcaactcttcgtgaaacctatggtgaaatggctgactgctgtgcaaaacaagaacctgagagaaatgaatgcttcttgcaacacaaagatgacaacccaaacctcccccgattggtgagaccagaggttgatgtgatgtgcactgcttttcatgacaatgaagagacatttttgaaaaaatacttatatgaaattgccagaagacatccttacttttatgccccggaactccttttctttgctaaaaggtataaagctgcttttacagaatgttgccaagctgctgataaagctgcctgcctgttgccaaagctcgatgaacttcgggatgaagggaaggcttcgtctgccaaacagagactcaagtgtgccagtctccaaaaatttggagaaagagctttcaaagcatgggcagtagctcgcctgagccagagatttcccaaagctgagtttgcagaagtttccaagttagtgacagatcttaccaaagtccacacggaatgctgccatggagatctgcttgaatgtgctgatgacagggcggaccttgccaagtatatctgtgaaaatcaagattcgatctccagtaaactgaaggaatgctgtgaaaaacctctgttggaaaaatcccactgcattgccgaagtggaaaatgatgagatgcctgctgacttgccttcattagctgctgattttgttgaaagtaaggatgtttgcaaaaactatgctgaggcaaaggatgtcttcctgggcatgtttttgtatgaatatgcaagaaggcatcctgattactctgtcgtgctgctgctgagacttgccaagacatatgaaaccactctagagaagtgctgtgccgctgcagatcctcatgaatgctatgccaaagtgttcgatgaatttaaacctcttgtggaagagcctcagaatttaatcaaacaaaattgtgagctttttgagcagcttggagagtacaaattccagaatgcgctattagttcgttacaccaagaaagtaccccaagtgtcaactccaactcttgtagaggtctcaagaaacctaggaaaagtgggcagcaaatgttgtaaacatcctgaagcaaaaagaatgccctgtgcagaagactatctatccgtggtcctgaaccagttatgtgtgttgcatgagaaaacgccagtaagtgacagagtcaccaaatgctgcacagaatccttggtgaacaggcgaccatgcttttcagctctggaagtcgatgaaacatacgttcccaaagagtttaatgctgaaacattcaccttccatgcagatatatgcacactttctgagaaggagagacaaatcaagaaacaaactgcacttgttgagctcgtgaaacacaagcccaaggcaacaaaagagcaactgaaagctgttatggatgatttcgcagcttttgtagagaagtgctgcaaggctgacgataaggagacctgctttgccgaggagggtaaaaaacttgttgctgcaagtcaagctgccttaggcttataa

SEQ ID NO: 16 - protein, 1009 aa, 人工序列（Artificial Sequence）
  CRIg-FH-HSA蛋白序列
GRPILEVPESVTGPWKGDVNLPCTYDPLQGYTQVLVKWLVQRGSDPVTIFLRDSSGDHIQQAKYQGRLHVSHKVPGDVSLQLSTLEMDDRSHYTCEVTWQTPDGNQVVRDKITELRVQKEDCNELPPRRNTEILTGSWSDQTYPEGTQAIYKCRPGYRSLGNVIMVCRKGEWVALNPLRKCQKRPCGHPGDTPFGTFTLTGGNVFEYGVKAVYTCNEGYQLLGEINYRECDTDGWTNDIPICEVVKCLPVTAPENGKIVSSAMEPDREYHFGQAVRFVCNSGYKIEGDEEMHCSDDGFWSKEKPKCVEISCKSPDVINGSPISQKIIYKENERFQYKCNMGYEYSERGDAVCTESGWRPLPSCEEKSCDNPYIPNGDYSPLRIKHRTGDEITYQCRNGFYPATRGNTAKCTSTGWIPAPRCTLKDAHKSEVAHRFKDLGEENFKALVLIAFAQYLQQCPFEDHVKLVNEVTEFAKTCVADESAENCDKSLHTLFGDKLCTVATLRETYGEMADCCAKQEPERNECFLQHKDDNPNLPRLVRPEVDVMCTAFHDNEETFLKKYLYEIARRHPYFYAPELLFFAKRYKAAFTECCQAADKAACLLPKLDELRDEGKASSAKQRLKCASLQKFGERAFKAWAVARLSQRFPKAEFAEVSKLVTDLTKVHTECCHGDLLECADDRADLAKYICENQDSISSKLKECCEKPLLEKSHCIAEVENDEMPADLPSLAADFVESKDVCKNYAEAKDVFLGMFLYEYARRHPDYSVVLLLRLAKTYETTLEKCCAAADPHECYAKVFDEFKPLVEEPQNLIKQNCELFEQLGEYKFQNALLVRYTKKVPQVSTPTLVEVSRNLGKVGSKCCKHPEAKRMPCAEDYLSVVLNQLCVLHEKTPVSDRVTKCCTESLVNRRPCFSALEVDETYVPKEFNAETFTFHADICTLSEKERQIKKQTALVELVKHKPKATKEQLKAVMDDFAAFVEKCCKADDKETCFAEEGKKLVAASQAALGL

SEQ ID NO: 17 - DNA, 1041 bp, 人工序列（Artificial Sequence）
  CD55核酸序列
gactgtggccttcccccagatgtacctaatgcccagccagctttggaaggccgtacaagttttcccgaggatactgtaataacgtacaaatgtgaagaaagctttgtgaaaattcctggcgagaaggactcagtgatctgccttaagggcagtcaatggtcagatattgaagagttctgcaatcgtagctgcgaggtgccaacaaggctaaattctgcatccctcaaacagccttatatcactcagaattattttccagtcggtactgttgtggaatatgagtgccgtccaggttacagaagagaaccttctctatcaccaaaactaacttgccttcagaatttaaaatggtccacagcagtcgaattttgtaaaaagaaatcatgccctaatccgggagaaatacgaaatggtcagattgatgtaccaggtggcatattatttggtgcaaccatctccttctcatgtaacacagggtacaaattatttggctcgacttctagtttttgtcttatttcaggcagctctgtccagtggagtgacccgttgccagagtgcagagaaatttattgtccagcaccaccacaaattgacaatggaataattcaaggggaacgtgaccattatggatatagacagtctgtaacgtatgcatgtaataaaggattcaccatgattggagagcactctatttattgtactgtgaataatgatgaaggagagtggagtggcccaccacctgaatgcagaggaaaatctctaacttccaaggtcccaccaacagttcagaaacctaccacagtaaatgttccaactacagaagtctcaccaacttctcagaaaaccaccacaaaaaccaccacaccaaatgctcaagcaacacggagtacacctgtttccaggacaaccaagcattttcatgaaacaaccccaaataaaggaagtggaaccacttcaggtactacccgtcttctatctgggcacacgtgtttcacgttgacaggtttgcttgggacgctagtaaccatgggcttgctgact

SEQ ID NO: 18 - protein, 347 aa, 人工序列（Artificial Sequence）
  CD55蛋白序列
DCGLPPDVPNAQPALEGRTSFPEDTVITYKCEESFVKIPGEKDSVICLKGSQWSDIEEFCNRSCEVPTRLNSASLKQPYITQNYFPVGTVVEYECRPGYRREPSLSPKLTCLQNLKWSTAVEFCKKKSCPNPGEIRNGQIDVPGGILFGATISFSCNTGYKLFGSTSSFCLISGSSVQWSDPLPECREIYCPAPPQIDNGIIQGERDHYGYRQSVTYACNKGFTMIGEHSIYCTVNNDEGEWSGPPPECRGKSLTSKVPPTVQKPTTVNVPTTEVSPTSQKTTTKTTTPNAQATRSTPVSRTTKHFHETTPNKGSGTTSGTTRLLSGHTCFTLTGLLGTLVTMGLLT

SEQ ID NO: 19 - DNA, 1074 bp, 人工序列（Artificial Sequence）
  CD46核酸序列
tgtgaggagccaccaacatttgaagctatggagctcattggtaaaccaaaaccctactatgagattggtgaacgagtagattataagtgtaaaaaaggatacttctatatacctcctcttgccacccatactatttgtgatcggaatcatacatggctacctgtctcagatgacgcctgttatagagaaacatgtccatatatacgggatcctttaaatggccaagcagtccctgcaaatgggacttacgagtttggttatcagatgcactttatttgtaatgagggttattacttaattggtgaagaaattctatattgtgaacttaaaggatcagtagcaatttggagcggtaagcccccaatatgtgaaaaggttttgtgtacaccacctccaaaaataaaaaatggaaaacacacctttagtgaagtagaagtatttgagtatcttgatgcagtaacttatagttgtgatcctgcacctggaccagatccattttcacttattggagagagcacgatttattgtggtgacaattcagtgtggagtcgtgctgctccagagtgtaaagtggtcaaatgtcgatttccagtagtcgaaaatggaaaacagatatcaggatttggaaaaaaattttactacaaagcaacagttatgtttgaatgcgataagggtttttacctcgatggcagcgacacaattgtctgtgacagtaacagtacttgggatcccccagttccaaagtgtcttaaagtgctgcctccatctagtacaaaacctccagctttgagtcattcagtgtcgacttcttccactacaaaatctccagcgtccagtgcctcaggtcctaggcctacttacaagcctccagtctcaaattatccaggatatcctaaacctgaggaaggaatacttgacagtttggatgtttgggtcattgctgtgattgttattgccatagttgttggagttgcagtaatttgtgttgtcccgtacagatatcttcaaaggaggaagaagaaaggcacatacctaactgatgagacccacagagaagtaaaatttacttctctc

SEQ ID NO: 20 - protein, 358 aa, 人工序列（Artificial Sequence）
  CD46蛋白序列
CEEPPTFEAMELIGKPKPYYEIGERVDYKCKKGYFYIPPLATHTICDRNHTWLPVSDDACYRETCPYIRDPLNGQAVPANGTYEFGYQMHFICNEGYYLIGEEILYCELKGSVAIWSGKPPICEKVLCTPPPKIKNGKHTFSEVEVFEYLDAVTYSCDPAPGPDPFSLIGESTIYCGDNSVWSRAAPECKVVKCRFPVVENGKQISGFGKKFYYKATVMFECDKGFYLDGSDTIVCDSNSTWDPPVPKCLKVLPPSSTKPPALSHSVSTSSTTKSPASSASGPRPTYKPPVSNYPGYPKPEEGILDSLDVWVIAVIVIAIVVGVAVICVVPYRYLQRRKKKGTYLTDETHREVKFTSL

SEQ ID NO: 21 - DNA, 309 bp, 人工序列（Artificial Sequence）
  CD59核酸序列
ctgcagtgctacaactgtcctaacccaactgctgactgcaaaacagccgtcaattgttcatctgattttgatgcgtgtctcattaccaaagctgggttacaagtgtataacaagtgttggaagtttgagcattgcaatttcaacgacgtcacaacccgcttgagggaaaatgagctaacgtactactgctgcaagaaggacctgtgtaactttaacgaacagcttgaaaatggtgggacatccttatcagagaaaacagttcttctgctggtgactccatttctggcagcagcctggagccttcatccc

SEQ ID NO: 22 - protein, 103 aa, 人工序列（Artificial Sequence）
  CD59蛋白序列
LQCYNCPNPTADCKTAVNCSSDFDACLITKAGLQVYNKCWKFEHCNFNDVTTRLRENELTYYCCKKDLCNFNEQLENGGTSLSEKTVLLLVTPFLAAAWSLHP

SEQ ID NO: 23 - DNA, 2076 bp, 人工序列（Artificial Sequence）
  CRIg-CD55-IgG4Fc核酸序列
atgggccgtcccatcctggaagtgccagagagtgtaacaggaccttggaaaggggatgtgaatcttccctgcacctatgaccccctgcaaggctacacccaagtcttggtgaagtggctggtacaacgtggctcagaccctgtcaccatctttctacgtgactcttctggagaccatatccagcaggcaaagtaccagggccgcctgcatgtgagccacaaggttccaggagatgtatccctccaattgagcaccctggagatggatgaccggagccactacacgtgtgaagtcacctggcagactcctgatggcaaccaagtcgtgagagataagattactgagctccgtgtccagaaagactgtggccttcccccagatgtacctaatgcccagccagctttggaaggccgtacaagttttcccgaggatactgtaataacgtacaaatgtgaagaaagctttgtgaaaattcctggcgagaaggactcagtgatctgccttaagggcagtcaatggtcagatattgaagagttctgcaatcgtagctgcgaggtgccaacaaggctaaattctgcatccctcaaacagccttatatcactcagaattattttccagtcggtactgttgtggaatatgagtgccgtccaggttacagaagagaaccttctctatcaccaaaactaacttgccttcagaatttaaaatggtccacagcagtcgaattttgtaaaaagaaatcatgccctaatccgggagaaatacgaaatggtcagattgatgtaccaggtggcatattatttggtgcaaccatctccttctcatgtaacacagggtacaaattatttggctcgacttctagtttttgtcttatttcaggcagctctgtccagtggagtgacccgttgccagagtgcagagaaatttattgtccagcaccaccacaaattgacaatggaataattcaaggggaacgtgaccattatggatatagacagtctgtaacgtatgcatgtaataaaggattcaccatgattggagagcactctatttattgtactgtgaataatgatgaaggagagtggagtggcccaccacctgaatgcagaggaaaatctctaacttccaaggtcccaccaacagttcagaaacctaccacagtaaatgttccaactacagaagtctcaccaacttctcagaaaaccaccacaaaaaccaccacaccaaatgctcaagcaacacggagtacacctgtttccaggacaaccaagcattttcatgaaacaaccccaaataaaggaagtggaaccacttcaggtactacccgtcttctatctgggcacacgtgtttcacgttgacaggtttgcttgggacgctagtaaccatgggcttgctgactcccccatgcccatcatgcccagcacctgagttcctggggggaccatcagtcttcctgttccccccaaaacccaaggacactctcatgatctcccggacccctgaggtcacgtgcgtggtggtggacgtgagccaggaagaccccgaggtccagttcaactggtacgtggatggcgtggaggtgcataatgccaagacaaagccgcgggaggagcagttcaacagcacgtaccgtgtggtcagcgtcctcaccgtcctgcaccaggactggctgaacggcaaggagtacaagtgcaaggtctccaacaaaggcctcccgtcctccatcgagaaaaccatctccaaagccaaagggcagccccgagagccacaggtgtacaccctgcccccatcccaggaggagatgaccaagaaccaggtcagcctgacctgcctggtcaaaggcttctaccccagcgacatcgccgtggagtgggagagcaatgggcagccggagaacaactacaagaccacgcctcccgtgctggactccgacggctccttcttcctctacagcaggctaaccgtggacaagagcaggtggcaggaggggaatgtcttctcatgctccgtgatgcatgaggctctgcacaaccactacacacagaagagcctctccctgtctctgggtaaataa

SEQ ID NO: 24 - protein, 691 aa, 人工序列（Artificial Sequence）
  CRIg-CD55-IgG4Fc蛋白序列
MGRPILEVPESVTGPWKGDVNLPCTYDPLQGYTQVLVKWLVQRGSDPVTIFLRDSSGDHIQQAKYQGRLHVSHKVPGDVSLQLSTLEMDDRSHYTCEVTWQTPDGNQVVRDKITELRVQKDCGLPPDVPNAQPALEGRTSFPEDTVITYKCEESFVKIPGEKDSVICLKGSQWSDIEEFCNRSCEVPTRLNSASLKQPYITQNYFPVGTVVEYECRPGYRREPSLSPKLTCLQNLKWSTAVEFCKKKSCPNPGEIRNGQIDVPGGILFGATISFSCNTGYKLFGSTSSFCLISGSSVQWSDPLPECREIYCPAPPQIDNGIIQGERDHYGYRQSVTYACNKGFTMIGEHSIYCTVNNDEGEWSGPPPECRGKSLTSKVPPTVQKPTTVNVPTTEVSPTSQKTTTKTTTPNAQATRSTPVSRTTKHFHETTPNKGSGTTSGTTRLLSGHTCFTLTGLLGTLVTMGLLTPPCPSCPAPEFLGGPSVFLFPPKPKDTLMISRTPEVTCVVVDVSQEDPEVQFNWYVDGVEVHNAKTKPREEQFNSTYRVVSVLTVLHQDWLNGKEYKCKVSNKGLPSSIEKTISKAKGQPREPQVYTLPPSQEEMTKNQVSLTCLVKGFYPSDIAVEWESNGQPENNYKTTPPVLDSDGSFFLYSRLTVDKSRWQEGNVFSCSVMHEALHNHYTQKSLSLSLGK

SEQ ID NO: 25 - DNA, 2109 bp, 人工序列（Artificial Sequence）
  CRIg-CD46-IgG4Fc核酸序列
atgggccgtcccatcctggaagtgccagagagtgtaacaggaccttggaaaggggatgtgaatcttccctgcacctatgaccccctgcaaggctacacccaagtcttggtgaagtggctggtacaacgtggctcagaccctgtcaccatctttctacgtgactcttctggagaccatatccagcaggcaaagtaccagggccgcctgcatgtgagccacaaggttccaggagatgtatccctccaattgagcaccctggagatggatgaccggagccactacacgtgtgaagtcacctggcagactcctgatggcaaccaagtcgtgagagataagattactgagctccgtgtccagaaatgtgaggagccaccaacatttgaagctatggagctcattggtaaaccaaaaccctactatgagattggtgaacgagtagattataagtgtaaaaaaggatacttctatatacctcctcttgccacccatactatttgtgatcggaatcatacatggctacctgtctcagatgacgcctgttatagagaaacatgtccatatatacgggatcctttaaatggccaagcagtccctgcaaatgggacttacgagtttggttatcagatgcactttatttgtaatgagggttattacttaattggtgaagaaattctatattgtgaacttaaaggatcagtagcaatttggagcggtaagcccccaatatgtgaaaaggttttgtgtacaccacctccaaaaataaaaaatggaaaacacacctttagtgaagtagaagtatttgagtatcttgatgcagtaacttatagttgtgatcctgcacctggaccagatccattttcacttattggagagagcacgatttattgtggtgacaattcagtgtggagtcgtgctgctccagagtgtaaagtggtcaaatgtcgatttccagtagtcgaaaatggaaaacagatatcaggatttggaaaaaaattttactacaaagcaacagttatgtttgaatgcgataagggtttttacctcgatggcagcgacacaattgtctgtgacagtaacagtacttgggatcccccagttccaaagtgtcttaaagtgctgcctccatctagtacaaaacctccagctttgagtcattcagtgtcgacttcttccactacaaaatctccagcgtccagtgcctcaggtcctaggcctacttacaagcctccagtctcaaattatccaggatatcctaaacctgaggaaggaatacttgacagtttggatgtttgggtcattgctgtgattgttattgccatagttgttggagttgcagtaatttgtgttgtcccgtacagatatcttcaaaggaggaagaagaaaggcacatacctaactgatgagacccacagagaagtaaaatttacttctctccccccatgcccatcatgcccagcacctgagttcctggggggaccatcagtcttcctgttccccccaaaacccaaggacactctcatgatctcccggacccctgaggtcacgtgcgtggtggtggacgtgagccaggaagaccccgaggtccagttcaactggtacgtggatggcgtggaggtgcataatgccaagacaaagccgcgggaggagcagttcaacagcacgtaccgtgtggtcagcgtcctcaccgtcctgcaccaggactggctgaacggcaaggagtacaagtgcaaggtctccaacaaaggcctcccgtcctccatcgagaaaaccatctccaaagccaaagggcagccccgagagccacaggtgtacaccctgcccccatcccaggaggagatgaccaagaaccaggtcagcctgacctgcctggtcaaaggcttctaccccagcgacatcgccgtggagtgggagagcaatgggcagccggagaacaactacaagaccacgcctcccgtgctggactccgacggctccttcttcctctacagcaggctaaccgtggacaagagcaggtggcaggaggggaatgtcttctcatgctccgtgatgcatgaggctctgcacaaccactacacacagaagagcctctccctgtctctgggtaaataa

SEQ ID NO: 26 - protein, 702 aa, 人工序列（Artificial Sequence）
  CRIg-CD46-IgG4Fc蛋白序列
MGRPILEVPESVTGPWKGDVNLPCTYDPLQGYTQVLVKWLVQRGSDPVTIFLRDSSGDHIQQAKYQGRLHVSHKVPGDVSLQLSTLEMDDRSHYTCEVTWQTPDGNQVVRDKITELRVQKCEEPPTFEAMELIGKPKPYYEIGERVDYKCKKGYFYIPPLATHTICDRNHTWLPVSDDACYRETCPYIRDPLNGQAVPANGTYEFGYQMHFICNEGYYLIGEEILYCELKGSVAIWSGKPPICEKVLCTPPPKIKNGKHTFSEVEVFEYLDAVTYSCDPAPGPDPFSLIGESTIYCGDNSVWSRAAPECKVVKCRFPVVENGKQISGFGKKFYYKATVMFECDKGFYLDGSDTIVCDSNSTWDPPVPKCLKVLPPSSTKPPALSHSVSTSSTTKSPASSASGPRPTYKPPVSNYPGYPKPEEGILDSLDVWVIAVIVIAIVVGVAVICVVPYRYLQRRKKKGTYLTDETHREVKFTSLPPCPSCPAPEFLGGPSVFLFPPKPKDTLMISRTPEVTCVVVDVSQEDPEVQFNWYVDGVEVHNAKTKPREEQFNSTYRVVSVLTVLHQDWLNGKEYKCKVSNKGLPSSIEKTISKAKGQPREPQVYTLPPSQEEMTKNQVSLTCLVKGFYPSDIAVEWESNGQPENNYKTTPPVLDSDGSFFLYSRLTVDKSRWQEGNVFSCSVMHEALHNHYTQKSLSLSLGK

SEQ ID NO: 27 - DNA, 1344 bp, 人工序列（Artificial Sequence）
  CRIg-CD59-IgG4Fc核酸序列
atgggccgtcccatcctggaagtgccagagagtgtaacaggaccttggaaaggggatgtgaatcttccctgcacctatgaccccctgcaaggctacacccaagtcttggtgaagtggctggtacaacgtggctcagaccctgtcaccatctttctacgtgactcttctggagaccatatccagcaggcaaagtaccagggccgcctgcatgtgagccacaaggttccaggagatgtatccctccaattgagcaccctggagatggatgaccggagccactacacgtgtgaagtcacctggcagactcctgatggcaaccaagtcgtgagagataagattactgagctccgtgtccagaaactgcagtgctacaactgtcctaacccaactgctgactgcaaaacagccgtcaattgttcatctgattttgatgcgtgtctcattaccaaagctgggttacaagtgtataacaagtgttggaagtttgagcattgcaatttcaacgacgtcacaacccgcttgagggaaaatgagctaacgtactactgctgcaagaaggacctgtgtaactttaacgaacagcttgaaaatggtgggacatccttatcagagaaaacagttcttctgctggtgactccatttctggcagcagcctggagccttcatccccccccatgcccatcatgcccagcacctgagttcctggggggaccatcagtcttcctgttccccccaaaacccaaggacactctcatgatctcccggacccctgaggtcacgtgcgtggtggtggacgtgagccaggaagaccccgaggtccagttcaactggtacgtggatggcgtggaggtgcataatgccaagacaaagccgcgggaggagcagttcaacagcacgtaccgtgtggtcagcgtcctcaccgtcctgcaccaggactggctgaacggcaaggagtacaagtgcaaggtctccaacaaaggcctcccgtcctccatcgagaaaaccatctccaaagccaaagggcagccccgagagccacaggtgtacaccctgcccccatcccaggaggagatgaccaagaaccaggtcagcctgacctgcctggtcaaaggcttctaccccagcgacatcgccgtggagtgggagagcaatgggcagccggagaacaactacaagaccacgcctcccgtgctggactccgacggctccttcttcctctacagcaggctaaccgtggacaagagcaggtggcaggaggggaatgtcttctcatgctccgtgatgcatgaggctctgcacaaccactacacacagaagagcctctccctgtctctgggtaaataa

SEQ ID NO: 28 - protein, 447 aa, 人工序列（Artificial Sequence）
  CRIg-CD59-IgG4Fc蛋白序列
MGRPILEVPESVTGPWKGDVNLPCTYDPLQGYTQVLVKWLVQRGSDPVTIFLRDSSGDHIQQAKYQGRLHVSHKVPGDVSLQLSTLEMDDRSHYTCEVTWQTPDGNQVVRDKITELRVQKLQCYNCPNPTADCKTAVNCSSDFDACLITKAGLQVYNKCWKFEHCNFNDVTTRLRENELTYYCCKKDLCNFNEQLENGGTSLSEKTVLLLVTPFLAAAWSLHPPPCPSCPAPEFLGGPSVFLFPPKPKDTLMISRTPEVTCVVVDVSQEDPEVQFNWYVDGVEVHNAKTKPREEQFNSTYRVVSVLTVLHQDWLNGKEYKCKVSNKGLPSSIEKTISKAKGQPREPQVYTLPPSQEEMTKNQVSLTCLVKGFYPSDIAVEWESNGQPENNYKTTPPVLDSDGSFFLYSRLTVDKSRWQEGNVFSCSVMHEALHNHYTQKSLSLSLGK

SEQ ID NO: 29 - DNA, 681 bp, 人工序列（Artificial Sequence）
  IgG1 Fc核酸序列
gacaaaactcacacatgcccaccgtgcccagcacctgaactcctggggggaccgtcagtcttcctcttccccccaaaacccaaggacaccctcatgatctcccggacccctgaggtcacatgcgtggtggtggacgtgagccacgaagaccctgaggtcaagttcaactggtacgtggacggcgtggaggtgcataatgccaagacaaagccgcgggaggagcagtacaacagcacgtaccgtgtggtcagcgtcctcaccgtcctgcaccaggactggctgaatggcaaggagtacaagtgcaaggtctccaacaaagccctcccagcccccatcgagaaaaccatctccaaagccaaagggcagccccgagaaccacaggtgtacaccctgcccccatcccgggaggagatgaccaagaaccaggtcagcctgacctgcctggtcaaaggcttctatcccagcgacatcgccgtggagtgggagagcaatgggcagccggagaacaactacaagaccacgcctcccgtgctggactccgacggctccttcttcctctacagcaagctcaccgtggacaagagcaggtggcagcaggggaacgtcttctcatgctccgtgatgcacgaggctctgcacaaccactacacgcagaagagcctctccctgtctccgggtaaa

SEQ ID NO: 30 - protein, 227 aa, 人工序列（Artificial Sequence）
  IgG1 Fc蛋白序列
DKTHTCPPCPAPELLGGPSVFLFPPKPKDTLMISRTPEVTCVVVDVSHEDPEVKFNWYVDGVEVHNAKTKPREEQYNSTYRVVSVLTVLHQDWLNGKEYKCKVSNKALPAPIEKTISKAKGQPREPQVYTLPPSREEMTKNQVSLTCLVKGFYPSDIAVEWESNGQPENNYKTTPPVLDSDGSFFLYSKLTVDKSRWQQGNVFSCSVMHEALHNHYTQKSLSLSPGK

SEQ ID NO: 31 - DNA, 681 bp, 人工序列（Artificial Sequence）
  Knob mutant核酸序列
gacaaaactcacacatgcccaccgtgcccagcacctgaactcgaggggggaccgtcagtcttcctcttccccccaaaacccaaggacaccctcatgatctcccggacccctgaggtcacatgcgtggtggtggacgtgagccacgaagaccctgaggtcaagttcaactggtacgtggacggcgtggaggtgcataatgccaagacaaagccgcgggaggagcagtacaacagcacgtaccgtgtggtcagcgtcctcaccgtcctgcaccaggactggctgaatggcaaggagtacaagtgcaaggtctccaacaaagccctcccagcccccatcgagaaaaccatctccaaagccaaagggcagccccgagaaccacaggtgtacaccctgcccccatcccgggaggagatgaccaagaaccaggtcagcctgtactgcctggtcaaaggcttctatcccagcgacatcgccgtggagtgggagagcaatgggcagccggagaacaactacaagaccacgcctcccgtgctggactccgacggctccttcttcctctacagcaagctcaccgtggacaagagcaggtggcagcaggggaacgtcttctcatgctccgtgatgcacgaggctctgcacaaccactacacgcagaagagcctctccctgtctccgggtaaa

SEQ ID NO: 32 - protein, 227 aa, 人工序列（Artificial Sequence）
  Knob mutant蛋白序列
DKTHTCPPCPAPELEGGPSVFLFPPKPKDTLMISRTPEVTCVVVDVSHEDPEVKFNWYVDGVEVHNAKTKPREEQYNSTYRVVSVLTVLHQDWLNGKEYKCKVSNKALPAPIEKTISKAKGQPREPQVYTLPPSREEMTKNQVSLYCLVKGFYPSDIAVEWESNGQPENNYKTTPPVLDSDGSFFLYSKLTVDKSRWQQGNVFSCSVMHEALHNHYTQKSLSLSPGK

SEQ ID NO: 33 - DNA, 681 bp, 人工序列（Artificial Sequence）
  Hole mutant核酸序列
gacaaaactcacacatgcccaccgtgcccagcacctgaactcgaggggggaccgtcagtcttcctcttccccccaaaacccaaggacaccctcatgatctcccggacccctgaggtcacatgcgtggtggtggacgtgagccacgaagaccctgaggtcaagttcaactggtacgtggacggcgtggaggtgcataatgccaagacaaagccgcgggaggagcagtacaacagcacgtaccgtgtggtcagcgtcctcaccgtcctgcaccaggactggctgaatggcaaggagtacaagtgcaaggtctccaacaaagccctcccagcccccatcgagaaaaccatctccaaagccaaagggcagccccgagaaccacaggtgtacaccctgcccccatcccgggaggagatgaccaagaaccaggtcagcctgacctgcctggtcaaaggcttctatcccagcgacatcgccgtggagtgggagagcaatgggcagccggagaacaactacaagaccacgcctcccgtgctggactccgacggctccttcttcctcaccagcaagctcaccgtggacaagagcaggtggcagcaggggaacgtcttctcatgctccgtgatgcacgaggctctgcacaaccactacacgcagaagagcctctccctgtctccgggtaaa

SEQ ID NO: 34 - protein, 227 aa, 人工序列（Artificial Sequence）
  Hole mutant蛋白序列
DKTHTCPPCPAPELEGGPSVFLFPPKPKDTLMISRTPEVTCVVVDVSHEDPEVKFNWYVDGVEVHNAKTKPREEQYNSTYRVVSVLTVLHQDWLNGKEYKCKVSNKALPAPIEKTISKAKGQPREPQVYTLPPSREEMTKNQVSLTCLVKGFYPSDIAVEWESNGQPENNYKTTPPVLDSDGSFFLTSKLTVDKSRWQQGNVFSCSVMHEALHNHYTQKSLSLSPGK

SEQ ID NO: 35 - DNA, 2118 bp, 人工序列（Artificial Sequence）
  CRIg-CD46-IgG1 Fc knob核酸序列
atgggccgtcccatcctggaagtgccagagagtgtaacaggaccttggaaaggggatgtgaatcttccctgcacctatgaccccctgcaaggctacacccaagtcttggtgaagtggctggtacaacgtggctcagaccctgtcaccatctttctacgtgactcttctggagaccatatccagcaggcaaagtaccagggccgcctgcatgtgagccacaaggttccaggagatgtatccctccaattgagcaccctggagatggatgaccggagccactacacgtgtgaagtcacctggcagactcctgatggcaaccaagtcgtgagagataagattactgagctccgtgtccagaaatgtgaggagccaccaacatttgaagctatggagctcattggtaaaccaaaaccctactatgagattggtgaacgagtagattataagtgtaaaaaaggatacttctatatacctcctcttgccacccatactatttgtgatcggaatcatacatggctacctgtctcagatgacgcctgttatagagaaacatgtccatatatacgggatcctttaaatggccaagcagtccctgcaaatgggacttacgagtttggttatcagatgcactttatttgtaatgagggttattacttaattggtgaagaaattctatattgtgaacttaaaggatcagtagcaatttggagcggtaagcccccaatatgtgaaaaggttttgtgtacaccacctccaaaaataaaaaatggaaaacacacctttagtgaagtagaagtatttgagtatcttgatgcagtaacttatagttgtgatcctgcacctggaccagatccattttcacttattggagagagcacgatttattgtggtgacaattcagtgtggagtcgtgctgctccagagtgtaaagtggtcaaatgtcgatttccagtagtcgaaaatggaaaacagatatcaggatttggaaaaaaattttactacaaagcaacagttatgtttgaatgcgataagggtttttacctcgatggcagcgacacaattgtctgtgacagtaacagtacttgggatcccccagttccaaagtgtcttaaagtgctgcctccatctagtacaaaacctccagctttgagtcattcagtgtcgacttcttccactacaaaatctccagcgtccagtgcctcaggtcctaggcctacttacaagcctccagtctcaaattatccaggatatcctaaacctgaggaaggaatacttgacagtttggatgtttgggtcattgctgtgattgttattgccatagttgttggagttgcagtaatttgtgttgtcccgtacagatatcttcaaaggaggaagaagaaaggcacatacctaactgatgagacccacagagaagtaaaatttacttctctcgacaaaactcacacatgcccaccgtgcccagcacctgaactcgaggggggaccgtcagtcttcctcttccccccaaaacccaaggacaccctcatgatctcccggacccctgaggtcacatgcgtggtggtggacgtgagccacgaagaccctgaggtcaagttcaactggtacgtggacggcgtggaggtgcataatgccaagacaaagccgcgggaggagcagtacaacagcacgtaccgtgtggtcagcgtcctcaccgtcctgcaccaggactggctgaatggcaaggagtacaagtgcaaggtctccaacaaagccctcccagcccccatcgagaaaaccatctccaaagccaaagggcagccccgagaaccacaggtgtacaccctgcccccatcccgggaggagatgaccaagaaccaggtcagcctgtactgcctggtcaaaggcttctatcccagcgacatcgccgtggagtgggagagcaatgggcagccggagaacaactacaagaccacgcctcccgtgctggactccgacggctccttcttcctctacagcaagctcaccgtggacaagagcaggtggcagcaggggaacgtcttctcatgctccgtgatgcacgaggctctgcacaaccactacacgcagaagagcctctccctgtctccgggtaaataa

SEQ ID NO: 36 - protein, 705 aa, 人工序列（Artificial Sequence）
  CRIg-CD46-IgG1 Fc knob蛋白序列
MGRPILEVPESVTGPWKGDVNLPCTYDPLQGYTQVLVKWLVQRGSDPVTIFLRDSSGDHIQQAKYQGRLHVSHKVPGDVSLQLSTLEMDDRSHYTCEVTWQTPDGNQVVRDKITELRVQKCEEPPTFEAMELIGKPKPYYEIGERVDYKCKKGYFYIPPLATHTICDRNHTWLPVSDDACYRETCPYIRDPLNGQAVPANGTYEFGYQMHFICNEGYYLIGEEILYCELKGSVAIWSGKPPICEKVLCTPPPKIKNGKHTFSEVEVFEYLDAVTYSCDPAPGPDPFSLIGESTIYCGDNSVWSRAAPECKVVKCRFPVVENGKQISGFGKKFYYKATVMFECDKGFYLDGSDTIVCDSNSTWDPPVPKCLKVLPPSSTKPPALSHSVSTSSTTKSPASSASGPRPTYKPPVSNYPGYPKPEEGILDSLDVWVIAVIVIAIVVGVAVICVVPYRYLQRRKKKGTYLTDETHREVKFTSLDKTHTCPPCPAPELEGGPSVFLFPPKPKDTLMISRTPEVTCVVVDVSHEDPEVKFNWYVDGVEVHNAKTKPREEQYNSTYRVVSVLTVLHQDWLNGKEYKCKVSNKALPAPIEKTISKAKGQPREPQVYTLPPSREEMTKNQVSLYCLVKGFYPSDIAVEWESNGQPENNYKTTPPVLDSDGSFFLYSKLTVDKSRWQQGNVFSCSVMHEALHNHYTQKSLSLSPGK

SEQ ID NO: 37 - DNA, 2085 bp, 人工序列（Artificial Sequence）
  CRIg-CD55-IgG1 Fc knob核酸序列
atgggccgtcccatcctggaagtgccagagagtgtaacaggaccttggaaaggggatgtgaatcttccctgcacctatgaccccctgcaaggctacacccaagtcttggtgaagtggctggtacaacgtggctcagaccctgtcaccatctttctacgtgactcttctggagaccatatccagcaggcaaagtaccagggccgcctgcatgtgagccacaaggttccaggagatgtatccctccaattgagcaccctggagatggatgaccggagccactacacgtgtgaagtcacctggcagactcctgatggcaaccaagtcgtgagagataagattactgagctccgtgtccagaaagactgtggccttcccccagatgtacctaatgcccagccagctttggaaggccgtacaagttttcccgaggatactgtaataacgtacaaatgtgaagaaagctttgtgaaaattcctggcgagaaggactcagtgatctgccttaagggcagtcaatggtcagatattgaagagttctgcaatcgtagctgcgaggtgccaacaaggctaaattctgcatccctcaaacagccttatatcactcagaattattttccagtcggtactgttgtggaatatgagtgccgtccaggttacagaagagaaccttctctatcaccaaaactaacttgccttcagaatttaaaatggtccacagcagtcgaattttgtaaaaagaaatcatgccctaatccgggagaaatacgaaatggtcagattgatgtaccaggtggcatattatttggtgcaaccatctccttctcatgtaacacagggtacaaattatttggctcgacttctagtttttgtcttatttcaggcagctctgtccagtggagtgacccgttgccagagtgcagagaaatttattgtccagcaccaccacaaattgacaatggaataattcaaggggaacgtgaccattatggatatagacagtctgtaacgtatgcatgtaataaaggattcaccatgattggagagcactctatttattgtactgtgaataatgatgaaggagagtggagtggcccaccacctgaatgcagaggaaaatctctaacttccaaggtcccaccaacagttcagaaacctaccacagtaaatgttccaactacagaagtctcaccaacttctcagaaaaccaccacaaaaaccaccacaccaaatgctcaagcaacacggagtacacctgtttccaggacaaccaagcattttcatgaaacaaccccaaataaaggaagtggaaccacttcaggtactacccgtcttctatctgggcacacgtgtttcacgttgacaggtttgcttgggacgctagtaaccatgggcttgctgactgacaaaactcacacatgcccaccgtgcccagcacctgaactcgaggggggaccgtcagtcttcctcttccccccaaaacccaaggacaccctcatgatctcccggacccctgaggtcacatgcgtggtggtggacgtgagccacgaagaccctgaggtcaagttcaactggtacgtggacggcgtggaggtgcataatgccaagacaaagccgcgggaggagcagtacaacagcacgtaccgtgtggtcagcgtcctcaccgtcctgcaccaggactggctgaatggcaaggagtacaagtgcaaggtctccaacaaagccctcccagcccccatcgagaaaaccatctccaaagccaaagggcagccccgagaaccacaggtgtacaccctgcccccatcccgggaggagatgaccaagaaccaggtcagcctgtactgcctggtcaaaggcttctatcccagcgacatcgccgtggagtgggagagcaatgggcagccggagaacaactacaagaccacgcctcccgtgctggactccgacggctccttcttcctctacagcaagctcaccgtggacaagagcaggtggcagcaggggaacgtcttctcatgctccgtgatgcacgaggctctgcacaaccactacacgcagaagagcctctccctgtctccgggtaaataa

SEQ ID NO: 38 - protein, 694 aa, 人工序列（Artificial Sequence）
  CRIg-CD55-IgG1 Fc knob蛋白序列
MGRPILEVPESVTGPWKGDVNLPCTYDPLQGYTQVLVKWLVQRGSDPVTIFLRDSSGDHIQQAKYQGRLHVSHKVPGDVSLQLSTLEMDDRSHYTCEVTWQTPDGNQVVRDKITELRVQKDCGLPPDVPNAQPALEGRTSFPEDTVITYKCEESFVKIPGEKDSVICLKGSQWSDIEEFCNRSCEVPTRLNSASLKQPYITQNYFPVGTVVEYECRPGYRREPSLSPKLTCLQNLKWSTAVEFCKKKSCPNPGEIRNGQIDVPGGILFGATISFSCNTGYKLFGSTSSFCLISGSSVQWSDPLPECREIYCPAPPQIDNGIIQGERDHYGYRQSVTYACNKGFTMIGEHSIYCTVNNDEGEWSGPPPECRGKSLTSKVPPTVQKPTTVNVPTTEVSPTSQKTTTKTTTPNAQATRSTPVSRTTKHFHETTPNKGSGTTSGTTRLLSGHTCFTLTGLLGTLVTMGLLTDKTHTCPPCPAPELEGGPSVFLFPPKPKDTLMISRTPEVTCVVVDVSHEDPEVKFNWYVDGVEVHNAKTKPREEQYNSTYRVVSVLTVLHQDWLNGKEYKCKVSNKALPAPIEKTISKAKGQPREPQVYTLPPSREEMTKNQVSLYCLVKGFYPSDIAVEWESNGQPENNYKTTPPVLDSDGSFFLYSKLTVDKSRWQQGNVFSCSVMHEALHNHYTQKSLSLSPGK

SEQ ID NO: 39 - DNA, 1959 bp, 人工序列（Artificial Sequence）
  CRIg-FH-IgG1 Fc hole核酸序列
atgggccgtcccatcctggaagtgccagagagtgtaacaggaccttggaaaggggatgtgaatcttccctgcacctatgaccccctgcaaggctacacccaagtcttggtgaagtggctggtacaacgtggctcagaccctgtcaccatctttctacgtgactcttctggagaccatatccagcaggcaaagtaccagggccgcctgcatgtgagccacaaggttccaggagatgtatccctccaattgagcaccctggagatggatgaccggagccactacacgtgtgaagtcacctggcagactcctgatggcaaccaagtcgtgagagataagattactgagctccgtgtccagaaagaagattgcaatgaacttcctccaagaagaaatacagaaattctgacaggttcctggtctgaccaaacatatccagaaggcacccaggctatctataaatgccgccctggatatagatctcttggaaatgtaataatggtatgcaggaagggagaatgggttgctcttaatccattaaggaaatgtcagaaaaggccctgtggacatcctggagatactccttttggtacttttacccttacaggaggaaatgtgtttgaatatggtgtaaaagctgtgtatacatgtaatgaggggtatcaattgctaggtgagattaattaccgtgaatgtgacacagatggatggaccaatgatattcctatatgtgaagttgtgaagtgtttaccagtgacagcaccagagaatggaaaaattgtcagtagtgcaatggaaccagatcgggaataccattttggacaagcagtacggtttgtatgtaactcaggctacaagattgaaggagatgaagaaatgcattgttcagacgatggtttttggagtaaagagaaaccaaagtgtgtggaaatttcatgcaaatccccagatgttataaatggatctcctatatctcagaagattatttataaggagaatgaacgatttcaatataaatgtaacatgggttatgaatacagtgaaagaggagatgctgtatgcactgaatctggatggcgtccgttgccttcatgtgaagaaaaatcatgtgataatccttatattccaaatggtgactactcacctttaaggattaaacacagaactggagatgaaatcacgtaccagtgtagaaatggtttttatcctgcaacccggggaaatacagcaaaatgcacaagtactggctggatacctgctccgagatgtaccttgaaagacaaaactcacacatgcccaccgtgcccagcacctgaactcgaggggggaccgtcagtcttcctcttccccccaaaacccaaggacaccctcatgatctcccggacccctgaggtcacatgcgtggtggtggacgtgagccacgaagaccctgaggtcaagttcaactggtacgtggacggcgtggaggtgcataatgccaagacaaagccgcgggaggagcagtacaacagcacgtaccgtgtggtcagcgtcctcaccgtcctgcaccaggactggctgaatggcaaggagtacaagtgcaaggtctccaacaaagccctcccagcccccatcgagaaaaccatctccaaagccaaagggcagccccgagaaccacaggtgtacaccctgcccccatcccgggaggagatgaccaagaaccaggtcagcctgacctgcctggtcaaaggcttctatcccagcgacatcgccgtggagtgggagagcaatgggcagccggagaacaactacaagaccacgcctcccgtgctggactccgacggctccttcttcctcaccagcaagctcaccgtggacaagagcaggtggcagcaggggaacgtcttctcatgctccgtgatgcacgaggctctgcacaaccactacacgcagaagagcctctccctgtctccgggtaaataa

SEQ ID NO: 40 - protein, 652 aa, 人工序列（Artificial Sequence）
  CRIg-FH-IgG1 Fc hole蛋白序列
MGRPILEVPESVTGPWKGDVNLPCTYDPLQGYTQVLVKWLVQRGSDPVTIFLRDSSGDHIQQAKYQGRLHVSHKVPGDVSLQLSTLEMDDRSHYTCEVTWQTPDGNQVVRDKITELRVQKEDCNELPPRRNTEILTGSWSDQTYPEGTQAIYKCRPGYRSLGNVIMVCRKGEWVALNPLRKCQKRPCGHPGDTPFGTFTLTGGNVFEYGVKAVYTCNEGYQLLGEINYRECDTDGWTNDIPICEVVKCLPVTAPENGKIVSSAMEPDREYHFGQAVRFVCNSGYKIEGDEEMHCSDDGFWSKEKPKCVEISCKSPDVINGSPISQKIIYKENERFQYKCNMGYEYSERGDAVCTESGWRPLPSCEEKSCDNPYIPNGDYSPLRIKHRTGDEITYQCRNGFYPATRGNTAKCTSTGWIPAPRCTLKDKTHTCPPCPAPELEGGPSVFLFPPKPKDTLMISRTPEVTCVVVDVSHEDPEVKFNWYVDGVEVHNAKTKPREEQYNSTYRVVSVLTVLHQDWLNGKEYKCKVSNKALPAPIEKTISKAKGQPREPQVYTLPPSREEMTKNQVSLTCLVKGFYPSDIAVEWESNGQPENNYKTTPPVLDSDGSFFLTSKLTVDKSRWQQGNVFSCSVMHEALHNHYTQKSLSLSPGK

SEQ ID NO: 41 - DNA, 1353 bp, 人工序列（Artificial Sequence）
  CRIg-CD59-IgG1 Fc hole核酸序列
atgggccgtcccatcctggaagtgccagagagtgtaacaggaccttggaaaggggatgtgaatcttccctgcacctatgaccccctgcaaggctacacccaagtcttggtgaagtggctggtacaacgtggctcagaccctgtcaccatctttctacgtgactcttctggagaccatatccagcaggcaaagtaccagggccgcctgcatgtgagccacaaggttccaggagatgtatccctccaattgagcaccctggagatggatgaccggagccactacacgtgtgaagtcacctggcagactcctgatggcaaccaagtcgtgagagataagattactgagctccgtgtccagaaactgcagtgctacaactgtcctaacccaactgctgactgcaaaacagccgtcaattgttcatctgattttgatgcgtgtctcattaccaaagctgggttacaagtgtataacaagtgttggaagtttgagcattgcaatttcaacgacgtcacaacccgcttgagggaaaatgagctaacgtactactgctgcaagaaggacctgtgtaactttaacgaacagcttgaaaatggtgggacatccttatcagagaaaacagttcttctgctggtgactccatttctggcagcagcctggagccttcatcccgacaaaactcacacatgcccaccgtgcccagcacctgaactcgaggggggaccgtcagtcttcctcttccccccaaaacccaaggacaccctcatgatctcccggacccctgaggtcacatgcgtggtggtggacgtgagccacgaagaccctgaggtcaagttcaactggtacgtggacggcgtggaggtgcataatgccaagacaaagccgcgggaggagcagtacaacagcacgtaccgtgtggtcagcgtcctcaccgtcctgcaccaggactggctgaatggcaaggagtacaagtgcaaggtctccaacaaagccctcccagcccccatcgagaaaaccatctccaaagccaaagggcagccccgagaaccacaggtgtacaccctgcccccatcccgggaggagatgaccaagaaccaggtcagcctgacctgcctggtcaaaggcttctatcccagcgacatcgccgtggagtgggagagcaatgggcagccggagaacaactacaagaccacgcctcccgtgctggactccgacggctccttcttcctcaccagcaagctcaccgtggacaagagcaggtggcagcaggggaacgtcttctcatgctccgtgatgcacgaggctctgcacaaccactacacgcagaagagcctctccctgtctccgggtaaataa

SEQ ID NO: 42 - protein, 450 aa, 人工序列（Artificial Sequence）
  CRIg-CD59-IgG1 Fc hole蛋白序列
MGRPILEVPESVTGPWKGDVNLPCTYDPLQGYTQVLVKWLVQRGSDPVTIFLRDSSGDHIQQAKYQGRLHVSHKVPGDVSLQLSTLEMDDRSHYTCEVTWQTPDGNQVVRDKITELRVQKLQCYNCPNPTADCKTAVNCSSDFDACLITKAGLQVYNKCWKFEHCNFNDVTTRLRENELTYYCCKKDLCNFNEQLENGGTSLSEKTVLLLVTPFLAAAWSLHPDKTHTCPPCPAPELEGGPSVFLFPPKPKDTLMISRTPEVTCVVVDVSHEDPEVKFNWYVDGVEVHNAKTKPREEQYNSTYRVVSVLTVLHQDWLNGKEYKCKVSNKALPAPIEKTISKAKGQPREPQVYTLPPSREEMTKNQVSLTCLVKGFYPSDIAVEWESNGQPENNYKTTPPVLDSDGSFFLTSKLTVDKSRWQQGNVFSCSVMHEALHNHYTQKSLSLSPGK

SEQ ID NO: 43 - DNA, 45 bp, 人工序列（Artificial Sequence）
  连接子1核酸序列
ggcggaggtggatctggcggaggtggatctggcggaggtggatct

SEQ ID NO: 44 - protein, 15 aa, 人工序列（Artificial Sequence）
  连接子1蛋白序列
GGGGSGGGGSGGGGS

SEQ ID NO: 45 - DNA, 24 bp, 人工序列（Artificial Sequence）
  连接子2核酸序列
ggcggaggtggaggcggaggtgga

SEQ ID NO: 46 - protein, 8 aa, 人工序列（Artificial Sequence）
  连接子2蛋白序列
GGGGGGGG

SEQ ID NO: 47 - DNA, 45 bp, 人工序列（Artificial Sequence）
  连接子3核酸序列
gaagctgccgcaaaggaagctgccgcaaaggaagctgccgcaaag

SEQ ID NO: 48 - protein, 15 aa, 人工序列（Artificial Sequence）
  连接子3蛋白序列
EAAAKEAAAKEAAAK

SEQ ID NO: 49 - DNA, 51 bp, 人工序列（Artificial Sequence）
  连接子4核酸序列
gttagtcaaacttctaaattaactcgtgccgagacagttttccctgatgtt

SEQ ID NO: 50 - protein, 17 aa, 人工序列（Artificial Sequence）
  连接子4蛋白序列
VSQTSKLTRAETVFPDV

SEQ ID NO: 51 - DNA, 1272 bp, 人工序列（Artificial Sequence）
  CRIg-FH的核酸序列
ggccgtcccatcctggaagtgccagagagtgtaacaggaccttggaaaggggatgtgaatcttccctgcacctatgaccccctgcaaggctacacccaagtcttggtgaagtggctggtacaacgtggctcagaccctgtcaccatctttctacgtgactcttctggagaccatatccagcaggcaaagtaccagggccgcctgcatgtgagccacaaggttccaggagatgtatccctccaattgagcaccctggagatggatgaccggagccactacacgtgtgaagtcacctggcagactcctgatggcaaccaagtcgtgagagataagattactgagctccgtgtccagaaagaagattgcaatgaacttcctccaagaagaaatacagaaattctgacaggttcctggtctgaccaaacatatccagaaggcacccaggctatctataaatgccgccctggatatagatctcttggaaatgtaataatggtatgcaggaagggagaatgggttgctcttaatccattaaggaaatgtcagaaaaggccctgtggacatcctggagatactccttttggtacttttacccttacaggaggaaatgtgtttgaatatggtgtaaaagctgtgtatacatgtaatgaggggtatcaattgctaggtgagattaattaccgtgaatgtgacacagatggatggaccaatgatattcctatatgtgaagttgtgaagtgtttaccagtgacagcaccagagaatggaaaaattgtcagtagtgcaatggaaccagatcgggaataccattttggacaagcagtacggtttgtatgtaactcaggctacaagattgaaggagatgaagaaatgcattgttcagacgatggtttttggagtaaagagaaaccaaagtgtgtggaaatttcatgcaaatccccagatgttataaatggatctcctatatctcagaagattatttataaggagaatgaacgatttcaatataaatgtaacatgggttatgaatacagtgaaagaggagatgctgtatgcactgaatctggatggcgtccgttgccttcatgtgaagaaaaatcatgtgataatccttatattccaaatggtgactactcacctttaaggattaaacacagaactggagatgaaatcacgtaccagtgtagaaatggtttttatcctgcaacccggggaaatacagcaaaatgcacaagtactggctggatacctgctccgagatgtaccttgaaa

SEQ ID NO: 52 - protein, 424 aa, 人工序列（Artificial Sequence）
  CRIg-FH的蛋白序列
GRPILEVPESVTGPWKGDVNLPCTYDPLQGYTQVLVKWLVQRGSDPVTIFLRDSSGDHIQQAKYQGRLHVSHKVPGDVSLQLSTLEMDDRSHYTCEVTWQTPDGNQVVRDKITELRVQKEDCNELPPRRNTEILTGSWSDQTYPEGTQAIYKCRPGYRSLGNVIMVCRKGEWVALNPLRKCQKRPCGHPGDTPFGTFTLTGGNVFEYGVKAVYTCNEGYQLLGEINYRECDTDGWTNDIPICEVVKCLPVTAPENGKIVSSAMEPDREYHFGQAVRFVCNSGYKIEGDEEMHCSDDGFWSKEKPKCVEISCKSPDVINGSPISQKIIYKENERFQYKCNMGYEYSERGDAVCTESGWRPLPSCEEKSCDNPYIPNGDYSPLRIKHRTGDEITYQCRNGFYPATRGNTAKCTSTGWIPAPRCTLK

SEQ ID NO: 53 - DNA, 1032 bp, 人工序列（Artificial Sequence）
  CRIg-IgG4 Fc核酸序列
ggccgtcccatcctggaagtgccagagagtgtaacaggaccttggaaaggggatgtgaatcttccctgcacctatgaccccctgcaaggctacacccaagtcttggtgaagtggctggtacaacgtggctcagaccctgtcaccatctttctacgtgactcttctggagaccatatccagcaggcaaagtaccagggccgcctgcatgtgagccacaaggttccaggagatgtatccctccaattgagcaccctggagatggatgaccggagccactacacgtgtgaagtcacctggcagactcctgatggcaaccaagtcgtgagagataagattactgagctccgtgtccagaaacccccatgcccatcatgcccagcacctgagttcctggggggaccatcagtcttcctgttccccccaaaacccaaggacactctcatgatctcccggacccctgaggtcacgtgcgtggtggtggacgtgagccaggaagaccccgaggtccagttcaactggtacgtggatggcgtggaggtgcataatgccaagacaaagccgcgggaggagcagttcaacagcacgtaccgtgtggtcagcgtcctcaccgtcctgcaccaggactggctgaacggcaaggagtacaagtgcaaggtctccaacaaaggcctcccgtcctccatcgagaaaaccatctccaaagccaaagggcagccccgagagccacaggtgtacaccctgcccccatcccaggaggagatgaccaagaaccaggtcagcctgacctgcctggtcaaaggcttctaccccagcgacatcgccgtggagtgggagagcaatgggcagccggagaacaactacaagaccacgcctcccgtgctggactccgacggctccttcttcctctacagcaggctaaccgtggacaagagcaggtggcaggaggggaatgtcttctcatgctccgtgatgcatgaggctctgcacaaccactacacacagaagagcctctccctgtctctgggtaaataa

SEQ ID NO: 54 - protein, 343 aa, 人工序列（Artificial Sequence）
  CRIg-IgG4 Fc蛋白序列
GRPILEVPESVTGPWKGDVNLPCTYDPLQGYTQVLVKWLVQRGSDPVTIFLRDSSGDHIQQAKYQGRLHVSHKVPGDVSLQLSTLEMDDRSHYTCEVTWQTPDGNQVVRDKITELRVQKPPCPSCPAPEFLGGPSVFLFPPKPKDTLMISRTPEVTCVVVDVSQEDPEVQFNWYVDGVEVHNAKTKPREEQFNSTYRVVSVLTVLHQDWLNGKEYKCKVSNKGLPSSIEKTISKAKGQPREPQVYTLPPSQEEMTKNQVSLTCLVKGFYPSDIAVEWESNGQPENNYKTTPPVLDSDGSFFLYSRLTVDKSRWQEGNVFSCSVMHEALHNHYTQKSLSLSLGK

SEQ ID NO: 55 - DNA, 1590 bp, 人工序列（Artificial Sequence）
  FH-IgG4 Fc 核酸序列
gaagattgcaatgaacttcctccaagaagaaatacagaaattctgacaggttcctggtctgaccaaacatatccagaaggcacccaggctatctataaatgccgccctggatatagatctcttggaaatgtaataatggtatgcaggaagggagaatgggttgctcttaatccattaaggaaatgtcagaaaaggccctgtggacatcctggagatactccttttggtacttttacccttacaggaggaaatgtgtttgaatatggtgtaaaagctgtgtatacatgtaatgaggggtatcaattgctaggtgagattaattaccgtgaatgtgacacagatggatggaccaatgatattcctatatgtgaagttgtgaagtgtttaccagtgacagcaccagagaatggaaaaattgtcagtagtgcaatggaaccagatcgggaataccattttggacaagcagtacggtttgtatgtaactcaggctacaagattgaaggagatgaagaaatgcattgttcagacgatggtttttggagtaaagagaaaccaaagtgtgtggaaatttcatgcaaatccccagatgttataaatggatctcctatatctcagaagattatttataaggagaatgaacgatttcaatataaatgtaacatgggttatgaatacagtgaaagaggagatgctgtatgcactgaatctggatggcgtccgttgccttcatgtgaagaaaaatcatgtgataatccttatattccaaatggtgactactcacctttaaggattaaacacagaactggagatgaaatcacgtaccagtgtagaaatggtttttatcctgcaacccggggaaatacagcaaaatgcacaagtactggctggatacctgctccgagatgtaccttgaaacccccatgcccatcatgcccagcacctgagttcctggggggaccatcagtcttcctgttccccccaaaacccaaggacactctcatgatctcccggacccctgaggtcacgtgcgtggtggtggacgtgagccaggaagaccccgaggtccagttcaactggtacgtggatggcgtggaggtgcataatgccaagacaaagccgcgggaggagcagttcaacagcacgtaccgtgtggtcagcgtcctcaccgtcctgcaccaggactggctgaacggcaaggagtacaagtgcaaggtctccaacaaaggcctcccgtcctccatcgagaaaaccatctccaaagccaaagggcagccccgagagccacaggtgtacaccctgcccccatcccaggaggagatgaccaagaaccaggtcagcctgacctgcctggtcaaaggcttctaccccagcgacatcgccgtggagtgggagagcaatgggcagccggagaacaactacaagaccacgcctcccgtgctggactccgacggctccttcttcctctacagcaggctaaccgtggacaagagcaggtggcaggaggggaatgtcttctcatgctccgtgatgcatgaggctctgcacaaccactacacacagaagagcctctccctgtctctgggtaaataa

SEQ ID NO: 56 - protein, 529 aa, 人工序列（Artificial Sequence）
  FH-IgG4 Fc蛋白序列
EDCNELPPRRNTEILTGSWSDQTYPEGTQAIYKCRPGYRSLGNVIMVCRKGEWVALNPLRKCQKRPCGHPGDTPFGTFTLTGGNVFEYGVKAVYTCNEGYQLLGEINYRECDTDGWTNDIPICEVVKCLPVTAPENGKIVSSAMEPDREYHFGQAVRFVCNSGYKIEGDEEMHCSDDGFWSKEKPKCVEISCKSPDVINGSPISQKIIYKENERFQYKCNMGYEYSERGDAVCTESGWRPLPSCEEKSCDNPYIPNGDYSPLRIKHRTGDEITYQCRNGFYPATRGNTAKCTSTGWIPAPRCTLKPPCPSCPAPEFLGGPSVFLFPPKPKDTLMISRTPEVTCVVVDVSQEDPEVQFNWYVDGVEVHNAKTKPREEQFNSTYRVVSVLTVLHQDWLNGKEYKCKVSNKGLPSSIEKTISKAKGQPREPQVYTLPPSQEEMTKNQVSLTCLVKGFYPSDIAVEWESNGQPENNYKTTPPVLDSDGSFFLYSRLTVDKSRWQEGNVFSCSVMHEALHNHYTQKSLSLSLGK

SEQ ID NO: 57 - DNA, 1947 bp, 人工序列（Artificial Sequence）
  FH-CRIg-IgG4 Fc 核酸序列
gaagattgcaatgaacttcctccaagaagaaatacagaaattctgacaggttcctggtctgaccaaacatatccagaaggcacccaggctatctataaatgccgccctggatatagatctcttggaaatgtaataatggtatgcaggaagggagaatgggttgctcttaatccattaaggaaatgtcagaaaaggccctgtggacatcctggagatactccttttggtacttttacccttacaggaggaaatgtgtttgaatatggtgtaaaagctgtgtatacatgtaatgaggggtatcaattgctaggtgagattaattaccgtgaatgtgacacagatggatggaccaatgatattcctatatgtgaagttgtgaagtgtttaccagtgacagcaccagagaatggaaaaattgtcagtagtgcaatggaaccagatcgggaataccattttggacaagcagtacggtttgtatgtaactcaggctacaagattgaaggagatgaagaaatgcattgttcagacgatggtttttggagtaaagagaaaccaaagtgtgtggaaatttcatgcaaatccccagatgttataaatggatctcctatatctcagaagattatttataaggagaatgaacgatttcaatataaatgtaacatgggttatgaatacagtgaaagaggagatgctgtatgcactgaatctggatggcgtccgttgccttcatgtgaagaaaaatcatgtgataatccttatattccaaatggtgactactcacctttaaggattaaacacagaactggagatgaaatcacgtaccagtgtagaaatggtttttatcctgcaacccggggaaatacagcaaaatgcacaagtactggctggatacctgctccgagatgtaccttgaaaggccgtcccatcctggaagtgccagagagtgtaacaggaccttggaaaggggatgtgaatcttccctgcacctatgaccccctgcaaggctacacccaagtcttggtgaagtggctggtacaacgtggctcagaccctgtcaccatctttctacgtgactcttctggagaccatatccagcaggcaaagtaccagggccgcctgcatgtgagccacaaggttccaggagatgtatccctccaattgagcaccctggagatggatgaccggagccactacacgtgtgaagtcacctggcagactcctgatggcaaccaagtcgtgagagataagattactgagctccgtgtccagaaacccccatgcccatcatgcccagcacctgagttcctggggggaccatcagtcttcctgttccccccaaaacccaaggacactctcatgatctcccggacccctgaggtcacgtgcgtggtggtggacgtgagccaggaagaccccgaggtccagttcaactggtacgtggatggcgtggaggtgcataatgccaagacaaagccgcgggaggagcagttcaacagcacgtaccgtgtggtcagcgtcctcaccgtcctgcaccaggactggctgaacggcaaggagtacaagtgcaaggtctccaacaaaggcctcccgtcctccatcgagaaaaccatctccaaagccaaagggcagccccgagagccacaggtgtacaccctgcccccatcccaggaggagatgaccaagaaccaggtcagcctgacctgcctggtcaaaggcttctaccccagcgacatcgccgtggagtgggagagcaatgggcagccggagaacaactacaagaccacgcctcccgtgctggactccgacggctccttcttcctctacagcaggctaaccgtggacaagagcaggtggcaggaggggaatgtcttctcatgctccgtgatgcatgaggctctgcacaaccactacacacagaagagcctctccctgtctctgggtaaataa

SEQ ID NO: 58 - protein, 648 aa, 人工序列（Artificial Sequence）
  FH-CRIg-IgG4 Fc蛋白序列
EDCNELPPRRNTEILTGSWSDQTYPEGTQAIYKCRPGYRSLGNVIMVCRKGEWVALNPLRKCQKRPCGHPGDTPFGTFTLTGGNVFEYGVKAVYTCNEGYQLLGEINYRECDTDGWTNDIPICEVVKCLPVTAPENGKIVSSAMEPDREYHFGQAVRFVCNSGYKIEGDEEMHCSDDGFWSKEKPKCVEISCKSPDVINGSPISQKIIYKENERFQYKCNMGYEYSERGDAVCTESGWRPLPSCEEKSCDNPYIPNGDYSPLRIKHRTGDEITYQCRNGFYPATRGNTAKCTSTGWIPAPRCTLKGRPILEVPESVTGPWKGDVNLPCTYDPLQGYTQVLVKWLVQRGSDPVTIFLRDSSGDHIQQAKYQGRLHVSHKVPGDVSLQLSTLEMDDRSHYTCEVTWQTPDGNQVVRDKITELRVQKPPCPSCPAPEFLGGPSVFLFPPKPKDTLMISRTPEVTCVVVDVSQEDPEVQFNWYVDGVEVHNAKTKPREEQFNSTYRVVSVLTVLHQDWLNGKEYKCKVSNKGLPSSIEKTISKAKGQPREPQVYTLPPSQEEMTKNQVSLTCLVKGFYPSDIAVEWESNGQPENNYKTTPPVLDSDGSFFLYSRLTVDKSRWQEGNVFSCSVMHEALHNHYTQKSLSLSLGK

SEQ ID NO: 59 - DNA, 1992 bp, 人工序列（Artificial Sequence）
  CRIg-L-FH-IgG4 Fc 核酸序列
ggccgtcccatcctggaagtgccagagagtgtaacaggaccttggaaaggggatgtgaatcttccctgcacctatgaccccctgcaaggctacacccaagtcttggtgaagtggctggtacaacgtggctcagaccctgtcaccatctttctacgtgactcttctggagaccatatccagcaggcaaagtaccagggccgcctgcatgtgagccacaaggttccaggagatgtatccctccaattgagcaccctggagatggatgaccggagccactacacgtgtgaagtcacctggcagactcctgatggcaaccaagtcgtgagagataagattactgagctccgtgtccagaaaggcggaggtggatctggcggaggtggatctggcggaggtggatctgaagattgcaatgaacttcctccaagaagaaatacagaaattctgacaggttcctggtctgaccaaacatatccagaaggcacccaggctatctataaatgccgccctggatatagatctcttggaaatgtaataatggtatgcaggaagggagaatgggttgctcttaatccattaaggaaatgtcagaaaaggccctgtggacatcctggagatactccttttggtacttttacccttacaggaggaaatgtgtttgaatatggtgtaaaagctgtgtatacatgtaatgaggggtatcaattgctaggtgagattaattaccgtgaatgtgacacagatggatggaccaatgatattcctatatgtgaagttgtgaagtgtttaccagtgacagcaccagagaatggaaaaattgtcagtagtgcaatggaaccagatcgggaataccattttggacaagcagtacggtttgtatgtaactcaggctacaagattgaaggagatgaagaaatgcattgttcagacgatggtttttggagtaaagagaaaccaaagtgtgtggaaatttcatgcaaatccccagatgttataaatggatctcctatatctcagaagattatttataaggagaatgaacgatttcaatataaatgtaacatgggttatgaatacagtgaaagaggagatgctgtatgcactgaatctggatggcgtccgttgccttcatgtgaagaaaaatcatgtgataatccttatattccaaatggtgactactcacctttaaggattaaacacagaactggagatgaaatcacgtaccagtgtagaaatggtttttatcctgcaacccggggaaatacagcaaaatgcacaagtactggctggatacctgctccgagatgtaccttgaaacccccatgcccatcatgcccagcacctgagttcctggggggaccatcagtcttcctgttccccccaaaacccaaggacactctcatgatctcccggacccctgaggtcacgtgcgtggtggtggacgtgagccaggaagaccccgaggtccagttcaactggtacgtggatggcgtggaggtgcataatgccaagacaaagccgcgggaggagcagttcaacagcacgtaccgtgtggtcagcgtcctcaccgtcctgcaccaggactggctgaacggcaaggagtacaagtgcaaggtctccaacaaaggcctcccgtcctccatcgagaaaaccatctccaaagccaaagggcagccccgagagccacaggtgtacaccctgcccccatcccaggaggagatgaccaagaaccaggtcagcctgacctgcctggtcaaaggcttctaccccagcgacatcgccgtggagtgggagagcaatgggcagccggagaacaactacaagaccacgcctcccgtgctggactccgacggctccttcttcctctacagcaggctaaccgtggacaagagcaggtggcaggaggggaatgtcttctcatgctccgtgatgcatgaggctctgcacaaccactacacacagaagagcctctccctgtctctgggtaaataa

SEQ ID NO: 60 - protein, 663 aa, 人工序列（Artificial Sequence）
  CRIg-L-FH-IgG4 Fc蛋白序列
GRPILEVPESVTGPWKGDVNLPCTYDPLQGYTQVLVKWLVQRGSDPVTIFLRDSSGDHIQQAKYQGRLHVSHKVPGDVSLQLSTLEMDDRSHYTCEVTWQTPDGNQVVRDKITELRVQKGGGGSGGGGSGGGGSEDCNELPPRRNTEILTGSWSDQTYPEGTQAIYKCRPGYRSLGNVIMVCRKGEWVALNPLRKCQKRPCGHPGDTPFGTFTLTGGNVFEYGVKAVYTCNEGYQLLGEINYRECDTDGWTNDIPICEVVKCLPVTAPENGKIVSSAMEPDREYHFGQAVRFVCNSGYKIEGDEEMHCSDDGFWSKEKPKCVEISCKSPDVINGSPISQKIIYKENERFQYKCNMGYEYSERGDAVCTESGWRPLPSCEEKSCDNPYIPNGDYSPLRIKHRTGDEITYQCRNGFYPATRGNTAKCTSTGWIPAPRCTLKPPCPSCPAPEFLGGPSVFLFPPKPKDTLMISRTPEVTCVVVDVSQEDPEVQFNWYVDGVEVHNAKTKPREEQFNSTYRVVSVLTVLHQDWLNGKEYKCKVSNKGLPSSIEKTISKAKGQPREPQVYTLPPSQEEMTKNQVSLTCLVKGFYPSDIAVEWESNGQPENNYKTTPPVLDSDGSFFLYSRLTVDKSRWQEGNVFSCSVMHEALHNHYTQKSLSLSLGK

SEQ ID NO: 61 - DNA, 762 bp, 人工序列（Artificial Sequence）
  CR1 CCP8-11的核酸序列
gatcattttctgtttgccaagttgaaaacccaaaccaatgcatctgactttcccattgggacatctttaaagtacgaatgccgtcctgagtactacgggaggccattctctatcacatgtctagataacctggtctggtcaagtcccaaagatgtctgtaaacgtaaatcatgtaaaactcctccagatccagtgaatggcatggtgcatgtgatcacagacatccaggttggatccagaatcaactattcttgtactacagggcaccgactcattggtcactcatctgctgaatgtatcctctcgggcaatgctgcccattggagcacgaagccgccaatttgtcaacgaattccttgtgggctaccccccaccatcgccaatggagatttcattagcaccaacagagagaattttcactatggatcagtggtgacctaccgctgcaatcctggaagcggagggagaaaggtgtttgagcttgtgggtgagccctccatatactgcaccagcaatgacgatcaagtgggcatctggagcggcccggcccctcagtgcattatacctaacaaatgcacgcctccaaatgtggaaaatggaatattggtatctgacaacagaagcttattttccttaaatgaagttgtggagtttaggtgtcagcctggctttgtcatgaaaggaccccgccgtgtgaagtgccaggccctgaacaaatgggagccggagctaccaagctgctccagggtatgtcagccacct

SEQ ID NO: 62 - protein, 254 aa, 人工序列（Artificial Sequence）
  CR1 CCP8-11的蛋白序列
DHFLFAKLKTQTNASDFPIGTSLKYECRPEYYGRPFSITCLDNLVWSSPKDVCKRKSCKTPPDPVNGMVHVITDIQVGSRINYSCTTGHRLIGHSSAECILSGNAAHWSTKPPICQRIPCGLPPTIANGDFISTNRENFHYGSVVTYRCNPGSGGRKVFELVGEPSIYCTSNDDQVGIWSGPAPQCIIPNKCTPPNVENGILVSDNRSLFSLNEVVEFRCQPGFVMKGPRRVKCQALNKWEPELPSCSRVCQPP

SEQ ID NO: 63 - DNA, 762 bp, 人工序列（Artificial Sequence）
  CR1 CCP15-18的核酸序列
gatcattttctgtttgccaagttgaaaacccaaaccaatgcatctgactttcccattgggacatctttaaagtacgaatgccgtcctgagtactacgggaggccattctctatcacatgtctagataacctggtctggtcaagtcccaaagatgtctgtaaacgtaaatcatgtaaaactcctccagatccagtgaatggcatggtgcatgtgatcacagacatccaggttggatccagaatcaactattcttgtactacagggcaccgactcattggtcactcatctgctgaatgtatcctctcaggcaatactgcccattggagcacgaagccgccaatttgtcaacgaattccttgtgggctacccccaaccatcgccaatggagatttcattagcaccaacagagagaattttcactatggatcagtggtgacctaccgctgcaatcttggaagcagagggagaaaggtgtttgagcttgtgggtgagccctccatatactgcaccagcaatgacgatcaagtgggcatctggagcggccccgcccctcagtgcattatacctaacaaatgcacgcctccaaatgtggaaaatggaatattggtatctgacaacagaagcttattttccttaaatgaagttgtggagtttaggtgtcagcctggctttgtcatgaaaggaccccgccgtgtgaagtgccaggccctgaacaaatgggagccagagttaccaagctgctccagggtgtgtcagccgcct

SEQ ID NO: 64 - protein, 254 aa, 人工序列（Artificial Sequence）
  CR1 CCP15-18的蛋白序列
DHFLFAKLKTQTNASDFPIGTSLKYECRPEYYGRPFSITCLDNLVWSSPKDVCKRKSCKTPPDPVNGMVHVITDIQVGSRINYSCTTGHRLIGHSSAECILSGNTAHWSTKPPICQRIPCGLPPTIANGDFISTNRENFHYGSVVTYRCNLGSRGRKVFELVGEPSIYCTSNDDQVGIWSGPAPQCIIPNKCTPPNVENGILVSDNRSLFSLNEVVEFRCQPGFVMKGPRRVKCQALNKWEPELPSCSRVCQPP

SEQ ID NO: 65 - DNA, 1794 bp, 人工序列（Artificial Sequence）
  CRIg-CR1(CCP8-11)-IgG4 Fc核酸序列
ggccgtcccatcctggaagtgccagagagtgtaacaggaccttggaaaggggatgtgaatcttccctgcacctatgaccccctgcaaggctacacccaagtcttggtgaagtggctggtacaacgtggctcagaccctgtcaccatctttctacgtgactcttctggagaccatatccagcaggcaaagtaccagggccgcctgcatgtgagccacaaggttccaggagatgtatccctccaattgagcaccctggagatggatgaccggagccactacacgtgtgaagtcacctggcagactcctgatggcaaccaagtcgtgagagataagattactgagctccgtgtccagaaagatcattttctgtttgccaagttgaaaacccaaaccaatgcatctgactttcccattgggacatctttaaagtacgaatgccgtcctgagtactacgggaggccattctctatcacatgtctagataacctggtctggtcaagtcccaaagatgtctgtaaacgtaaatcatgtaaaactcctccagatccagtgaatggcatggtgcatgtgatcacagacatccaggttggatccagaatcaactattcttgtactacagggcaccgactcattggtcactcatctgctgaatgtatcctctcgggcaatgctgcccattggagcacgaagccgccaatttgtcaacgaattccttgtgggctaccccccaccatcgccaatggagatttcattagcaccaacagagagaattttcactatggatcagtggtgacctaccgctgcaatcctggaagcggagggagaaaggtgtttgagcttgtgggtgagccctccatatactgcaccagcaatgacgatcaagtgggcatctggagcggcccggcccctcagtgcattatacctaacaaatgcacgcctccaaatgtggaaaatggaatattggtatctgacaacagaagcttattttccttaaatgaagttgtggagtttaggtgtcagcctggctttgtcatgaaaggaccccgccgtgtgaagtgccaggccctgaacaaatgggagccggagctaccaagctgctccagggtatgtcagccacctcccccatgcccatcatgcccagcacctgagttcctggggggaccatcagtcttcctgttccccccaaaacccaaggacactctcatgatctcccggacccctgaggtcacgtgcgtggtggtggacgtgagccaggaagaccccgaggtccagttcaactggtacgtggatggcgtggaggtgcataatgccaagacaaagccgcgggaggagcagttcaacagcacgtaccgtgtggtcagcgtcctcaccgtcctgcaccaggactggctgaacggcaaggagtacaagtgcaaggtctccaacaaaggcctcccgtcctccatcgagaaaaccatctccaaagccaaagggcagccccgagagccacaggtgtacaccctgcccccatcccaggaggagatgaccaagaaccaggtcagcctgacctgcctggtcaaaggcttctaccccagcgacatcgccgtggagtgggagagcaatgggcagccggagaacaactacaagaccacgcctcccgtgctggactccgacggctccttcttcctctacagcaggctaaccgtggacaagagcaggtggcaggaggggaatgtcttctcatgctccgtgatgcatgaggctctgcacaaccactacacacagaagagcctctccctgtctctgggtaaataa

SEQ ID NO: 66 - protein, 597 aa, 人工序列（Artificial Sequence）
  CRIg-CR1(CCP8-11)-IgG4 Fc蛋白序列
GRPILEVPESVTGPWKGDVNLPCTYDPLQGYTQVLVKWLVQRGSDPVTIFLRDSSGDHIQQAKYQGRLHVSHKVPGDVSLQLSTLEMDDRSHYTCEVTWQTPDGNQVVRDKITELRVQKDHFLFAKLKTQTNASDFPIGTSLKYECRPEYYGRPFSITCLDNLVWSSPKDVCKRKSCKTPPDPVNGMVHVITDIQVGSRINYSCTTGHRLIGHSSAECILSGNAAHWSTKPPICQRIPCGLPPTIANGDFISTNRENFHYGSVVTYRCNPGSGGRKVFELVGEPSIYCTSNDDQVGIWSGPAPQCIIPNKCTPPNVENGILVSDNRSLFSLNEVVEFRCQPGFVMKGPRRVKCQALNKWEPELPSCSRVCQPPPPCPSCPAPEFLGGPSVFLFPPKPKDTLMISRTPEVTCVVVDVSQEDPEVQFNWYVDGVEVHNAKTKPREEQFNSTYRVVSVLTVLHQDWLNGKEYKCKVSNKGLPSSIEKTISKAKGQPREPQVYTLPPSQEEMTKNQVSLTCLVKGFYPSDIAVEWESNGQPENNYKTTPPVLDSDGSFFLYSRLTVDKSRWQEGNVFSCSVMHEALHNHYTQKSLSLSLGK

SEQ ID NO: 67 - DNA, 1794 bp, 人工序列（Artificial Sequence）
  CRIg-CR1(CCP15-18)-IgG4 Fc核酸序列
ggccgtcccatcctggaagtgccagagagtgtaacaggaccttggaaaggggatgtgaatcttccctgcacctatgaccccctgcaaggctacacccaagtcttggtgaagtggctggtacaacgtggctcagaccctgtcaccatctttctacgtgactcttctggagaccatatccagcaggcaaagtaccagggccgcctgcatgtgagccacaaggttccaggagatgtatccctccaattgagcaccctggagatggatgaccggagccactacacgtgtgaagtcacctggcagactcctgatggcaaccaagtcgtgagagataagattactgagctccgtgtccagaaagatcattttctgtttgccaagttgaaaacccaaaccaatgcatctgactttcccattgggacatctttaaagtacgaatgccgtcctgagtactacgggaggccattctctatcacatgtctagataacctggtctggtcaagtcccaaagatgtctgtaaacgtaaatcatgtaaaactcctccagatccagtgaatggcatggtgcatgtgatcacagacatccaggttggatccagaatcaactattcttgtactacagggcaccgactcattggtcactcatctgctgaatgtatcctctcaggcaatactgcccattggagcacgaagccgccaatttgtcaacgaattccttgtgggctacccccaaccatcgccaatggagatttcattagcaccaacagagagaattttcactatggatcagtggtgacctaccgctgcaatcttggaagcagagggagaaaggtgtttgagcttgtgggtgagccctccatatactgcaccagcaatgacgatcaagtgggcatctggagcggccccgcccctcagtgcattatacctaacaaatgcacgcctccaaatgtggaaaatggaatattggtatctgacaacagaagcttattttccttaaatgaagttgtggagtttaggtgtcagcctggctttgtcatgaaaggaccccgccgtgtgaagtgccaggccctgaacaaatgggagccagagttaccaagctgctccagggtgtgtcagccgcctcccccatgcccatcatgcccagcacctgagttcctggggggaccatcagtcttcctgttccccccaaaacccaaggacactctcatgatctcccggacccctgaggtcacgtgcgtggtggtggacgtgagccaggaagaccccgaggtccagttcaactggtacgtggatggcgtggaggtgcataatgccaagacaaagccgcgggaggagcagttcaacagcacgtaccgtgtggtcagcgtcctcaccgtcctgcaccaggactggctgaacggcaaggagtacaagtgcaaggtctccaacaaaggcctcccgtcctccatcgagaaaaccatctccaaagccaaagggcagccccgagagccacaggtgtacaccctgcccccatcccaggaggagatgaccaagaaccaggtcagcctgacctgcctggtcaaaggcttctaccccagcgacatcgccgtggagtgggagagcaatgggcagccggagaacaactacaagaccacgcctcccgtgctggactccgacggctccttcttcctctacagcaggctaaccgtggacaagagcaggtggcaggaggggaatgtcttctcatgctccgtgatgcatgaggctctgcacaaccactacacacagaagagcctctccctgtctctgggtaaataa

SEQ ID NO: 68 - protein, 597 aa, 人工序列（Artificial Sequence）
  CRIg-CR1(CCP15-18)-IgG4 Fc蛋白序列
GRPILEVPESVTGPWKGDVNLPCTYDPLQGYTQVLVKWLVQRGSDPVTIFLRDSSGDHIQQAKYQGRLHVSHKVPGDVSLQLSTLEMDDRSHYTCEVTWQTPDGNQVVRDKITELRVQKDHFLFAKLKTQTNASDFPIGTSLKYECRPEYYGRPFSITCLDNLVWSSPKDVCKRKSCKTPPDPVNGMVHVITDIQVGSRINYSCTTGHRLIGHSSAECILSGNTAHWSTKPPICQRIPCGLPPTIANGDFISTNRENFHYGSVVTYRCNLGSRGRKVFELVGEPSIYCTSNDDQVGIWSGPAPQCIIPNKCTPPNVENGILVSDNRSLFSLNEVVEFRCQPGFVMKGPRRVKCQALNKWEPELPSCSRVCQPPPPCPSCPAPEFLGGPSVFLFPPKPKDTLMISRTPEVTCVVVDVSQEDPEVQFNWYVDGVEVHNAKTKPREEQFNSTYRVVSVLTVLHQDWLNGKEYKCKVSNKGLPSSIEKTISKAKGQPREPQVYTLPPSQEEMTKNQVSLTCLVKGFYPSDIAVEWESNGQPENNYKTTPPVLDSDGSFFLYSRLTVDKSRWQEGNVFSCSVMHEALHNHYTQKSLSLSLGK